European Patent Specification EP 3 551 197 B1, published November 22, 2023. Title: CHIMERIC TRANSCRIPTION FACTOR VARIANTS WITH AUGMENTED SENSITIVITY TO DRUG LIGAND INDUCTION OF TRANSGENE EXPRESSION IN MAMMMALIAN CELLS. Applicant: Seattle Children's Research Institute Jensen, Michael C. Ooi, Tracy Wei, Jia. The sequence listing filed with the application follows.

SEQUENCE LISTING (124 sequences)

SEQ ID NO: 1 - protein, 862 aa, Artificial Sequence
  chimeric transcription factor composed of human subunits
MVSKLSQLQTELLAALLESGLSKEALIQALGEPGPYLLAGEGPLDKGESCGGGRGELAELPNGLGETRGSEDETDDDGEDFTPPILKELENLSPEEAAHQKAVVETLLQEDPWRVAKMVKSYLQQHNIPQREVVDTTGLNQSHLSQHLNKGTPMKTQKRAALYTWYVRKQREVAQQFTHAGQGGLIEEPTGDELPTKKGRRNRFKWGPASQQILFQAYERQKNPSKEERETLVEECNRAECIQRGVSPSQAQGLGSNLVTEVRVYNWFANRRKEEAFRHKLSAGDMRAANLWPSPLMIKRSKKNSLALSLTADQMVSALLDAEPPILYSEYDPTRPFSEASMMGLLTNLADRELVHMINWAKRVPGFVDLTLHDQVHLLECAWLEILMIGLVWRSMEHPGKLLFAPNLLLDRNQGKCVEGMVEIFDMLLATSSRFRMMNLQGEEFVCLKSIILLNSGVYTFLSSTLKSLEEKDHIHRVLDKITDTLIHLMAKAGLTLQQQHQRLAQLLLILSHIRHMSNKRMEHLYSMKCKNVVPLYDLLLEMLDAHRLHAPTSRGGASVEETDQSHLATAGSTSSHSLQKYYITGEAEGFPATVEFQYLPDTDDRHRIEEKRKRTYETFKSIMKKSPFSGPTDPRPPPRRIAVPSRSSASVPKPAPQPYPFTSSLSTINYDEFPTMVFPSGQISQASALAPAPPQVLPQAPAPAPAPAMVSALAQAPAPVPVLAPGPPQAVAPPAPKPTQAGEGTLSEALLQLQFDDEDLGALLGNSTDPAVFTDLASVDNSEFQQLLNQGIPVAPHTTEPMLMEYPEAITRLVTGAQRPPDPAPAPLGAPGLPNGLLSGDEDFSSIADMDFSALLSQISS

SEQ ID NO: 2 - protein, 862 aa, Artificial Sequence
  HEA3 transcription factor with one point mutation in the p65 domain
MVSKLSQLQTELLAALLESGLSKEALIQALGEPGPYLLAGEGPLDKGESCGGGRGELAELPNGLGETRGSEDETDDDGEDFTPPILKELENLSPEEAAHQKAVVETLLQEDPWRVAKMVKSYLQQHNIPQREVVDTTGLNQSHLSQHLNKGTPMKTQKRAALYTWYVRKQREVAQQFTHAGQGGLIEEPTGDELPTKKGRRNRFKWGPASQQILFQAYERQKNPSKEERETLVEECNRAECIQRGVSPSQAQGLGSNLVTEVRVYNWFANRRKEEAFRHKLSAGDMRAANLWPSPLMIKRSKKNSLALSLTADQMVSALLDAEPPILYSEYDPTRPFSEASMMGLLTNLADRELVHMINWAKRVPGFVDLTLHDQVHLLECAWLEILMIGLVWRSMEHPGKLLFAPNLLLDRNQGKCVEGMVEIFDMLLATSSRFRMMNLQGEEFVCLKSIILLNSGVYTFLSSTLKSLEEKDHIHRVLDKITDTLIHLMAKAGLTLQQQHQRLAQLLLILSHIRHMSNKRMEHLYSMKCKNVVPLYDLLLEMLDAHRLHAPTSRGGASVEETDQSHLATAGSTSSHSLQKYYITGEAEGFPATVEFQYLPDTDDRHRIEEKRKRTYETFKSIMKKSPFSGPTDPRPPPRRIAVPSRSSASVPKPAPQPYPFTSSLSTINYDEFPTMVFPSGQISQASALAPAPPQVLPQAPAPAPAPAMVSALAQAPAPVPVLAPGPPQAVAPPAPKPTQAGEGTLSEALLQLQFDDEDLGALLGNSTDPAVFTDLASVDNSEFQQLLNQGIPVAPHTTEPMLMEYPEAITRLVTGAQRPPDPAPAPLGAPGLPNGLLSGDEDFESIADMDFSALLSQISS

SEQ ID NO: 3 - protein, 862 aa, Artificial Sequence
  HEA3 containing one point mutation in the p65 domain
MVSKLSQLQTELLAALLESGLSKEALIQALGEPGPYLLAGEGPLDKGESCGGGRGELAELPNGLGETRGSEDETDDDGEDFTPPILKELENLSPEEAAHQKAVVETLLQEDPWRVAKMVKSYLQQHNIPQREVVDTTGLNQSHLSQHLNKGTPMKTQKRAALYTWYVRKQREVAQQFTHAGQGGLIEEPTGDELPTKKGRRNRFKWGPASQQILFQAYERQKNPSKEERETLVEECNRAECIQRGVSPSQAQGLGSNLVTEVRVYNWFANRRKEEAFRHKLSAGDMRAANLWPSPLMIKRSKKNSLALSLTADQMVSALLDAEPPILYSEYDPTRPFSEASMMGLLTNLADRELVHMINWAKRVPGFVDLTLHDQVHLLECAWLEILMIGLVWRSMEHPGKLLFAPNLLLDRNQGKCVEGMVEIFDMLLATSSRFRMMNLQGEEFVCLKSIILLNSGVYTFLSSTLKSLEEKDHIHRVLDKITDTLIHLMAKAGLTLQQQHQRLAQLLLILSHIRHMSNKRMEHLYSMKCKNVVPLYDLLLEMLDAHRLHAPTSRGGASVEETDQSHLATAGSTSSHSLQKYYITGEAEGFPATVEFQYLPDTDDRHRIEEKRKRTYETFQSIMKKSPFSGPTDPRPPPRRIAVPSRSSASVPKPAPQPYPFTSSLSTINYDEFPTMVFPSGQISQASALAPAPPQVLPQAPAPAPAPAMVSALAQAPAPVPVLAPGPPQAVAPPAPKPTQAGEGTLSEALLQLQFDDEDLGALLGNSTDPAVFTDLASVDNSEFQQLLNQGIPVAPHTTEPMLMEYPEAITRLVTGAQRPPDPAPAPLGAPGLPNGLLSGDEDFSSIADMDFSALLSQISS

SEQ ID NO: 4 - protein, 862 aa, Artificial Sequence
  HEA4 comprising at least three mutations
MVSKLSQLQTELLAALLESGLSKEALIQALGEPGPYLLAGEGPLDKGESCGGGRGELAELPNGLGETRGSEDETDDDGEDFTPPILKELENLSPEEAAHQKAVVETLLQEDPWRVAKMVKSYLQQHNIPQREVVDTTGLNQSHLSQHLNKGTPMKTQKRAALYTWYVRKQREVAQQFTHAGQGGLIEEPTGDELPTKKGRRNRFKWGPASQQILFQAYERQKNPSKEERETLVEECNRAECIQRGVSPSQAQGLGSNLVTEVRVYNWFANRRKEEAFRHKLSAGDMRAANLWPSPLMIKRSKKNSLALSLTADQMVSALLDAEPPILYSEYDPTRPFSEASMMGLLTNLADRELVHMINWAKRVPGFVDLTLHDQVHLLECAWLEILMIGLVWRSMEHPVKLLFAPNLLLDRNQGKCVEGMVEIFDMLLATSSRFRMMNLQGEEFVCLKSIILLNSGVYTFLSSTLKSLEEKDHIHRVLDKITDTLIHLMAKAGLTLQQQHQRLAQLLLILSHIRHMSNKGMEHLYSMKCKNVVPLYDLLLEAADAHRLHAPTSRGGASVEETDQSHLATAGSTSSHSLQKYYITGEAEGFPATVEFQYLPDTDDRHRIEEKRKRTYETFKSIMKKSPFSGPTDPRPPPRRIAVPSRSSASVPKPAPQPYPFTSSLSTINYDEFPTMVFPSGQISQASALAPAPPQVLPQAPAPAPAPAMVSALAQAPAPVPVLAPGPPQAVAPPAPKPTQAGEGTLSEALLQLQFDDEDLGALLGNSTDPAVFTDLASVDNSEFQQLLNQGIPVAPHTTEPMLMEYPEAITRLVTGAQRPPDPAPAPLGAPGLPNGLLSGDEDFSSIADMDFSALLSQISS

SEQ ID NO: 5 - protein, 862 aa, Artificial Sequence
  HEA4 containing one point mutation in the p65 domain
MVSKLSQLQTELLAALLESGLSKEALIQALGEPGPYLLAGEGPLDKGESCGGGRGELAELPNGLGETRGSEDETDDDGEDFTPPILKELENLSPEEAAHQKAVVETLLQEDPWRVAKMVKSYLQQHNIPQREVVDTTGLNQSHLSQHLNKGTPMKTQKRAALYTWYVRKQREVAQQFTHAGQGGLIEEPTGDELPTKKGRRNRFKWGPASQQILFQAYERQKNPSKEERETLVEECNRAECIQRGVSPSQAQGLGSNLVTEVRVYNWFANRRKEEAFRHKLSAGDMRAANLWPSPLMIKRSKKNSLALSLTADQMVSALLDAEPPILYSEYDPTRPFSEASMMGLLTNLADRELVHMINWAKRVPGFVDLTLHDQVHLLECAWLEILMIGLVWRSMEHPVKLLFAPNLLLDRNQGKCVEGMVEIFDMLLATSSRFRMMNLQGEEFVCLKSIILLNSGVYTFLSSTLKSLEEKDHIHRVLDKITDTLIHLMAKAGLTLQQQHQRLAQLLLILSHIRHMSNKGMEHLYSMKCKNVVPLYDLLLEAADAHRLHAPTSRGGASVEETDQSHLATAGSTSSHSLQKYYITGEAEGFPATVEFQYLPDTDDRHRIEEKRKRTYETFKSIMKKSPFSGPTDPRPPPRRIAVPSRSSASVPKPAPQPYPFTSSLSTINYDEFPTMVFPSGQISQASALAPAPPQVLPQAPAPAPAPAMVSALAQAPAPVPVLAPGPPQAVAPPAPKPTQAGEGTLSEALLQLQFDDEDLGALLGNSTDPAVFTDLASVDNSEFQQLLNQGIPVAPHTTEPMLMEYPEAITRLVTGAQRPPDPAPAPLGAPGLPNGLLSGDEDFESIADMDFSALLSQISS

SEQ ID NO: 6 - protein, 862 aa, Artificial Sequence
  HEA4 containing one point mutation in the p65 domain
MVSKLSQLQTELLAALLESGLSKEALIQALGEPGPYLLAGEGPLDKGESCGGGRGELAELPNGLGETRGSEDETDDDGEDFTPPILKELENLSPEEAAHQKAVVETLLQEDPWRVAKMVKSYLQQHNIPQREVVDTTGLNQSHLSQHLNKGTPMKTQKRAALYTWYVRKQREVAQQFTHAGQGGLIEEPTGDELPTKKGRRNRFKWGPASQQILFQAYERQKNPSKEERETLVEECNRAECIQRGVSPSQAQGLGSNLVTEVRVYNWFANRRKEEAFRHKLSAGDMRAANLWPSPLMIKRSKKNSLALSLTADQMVSALLDAEPPILYSEYDPTRPFSEASMMGLLTNLADRELVHMINWAKRVPGFVDLTLHDQVHLLECAWLEILMIGLVWRSMEHPVKLLFAPNLLLDRNQGKCVEGMVEIFDMLLATSSRFRMMNLQGEEFVCLKSIILLNSGVYTFLSSTLKSLEEKDHIHRVLDKITDTLIHLMAKAGLTLQQQHQRLAQLLLILSHIRHMSNKGMEHLYSMKCKNVVPLYDLLLEAADAHRLHAPTSRGGASVEETDQSHLATAGSTSSHSLQKYYITGEAEGFPATVEFQYLPDTDDRHRIEEKRKRTYETFQSIMKKSPFSGPTDPRPPPRRIAVPSRSSASVPKPAPQPYPFTSSLSTINYDEFPTMVFPSGQISQASALAPAPPQVLPQAPAPAPAPAMVSALAQAPAPVPVLAPGPPQAVAPPAPKPTQAGEGTLSEALLQLQFDDEDLGALLGNSTDPAVFTDLASVDNSEFQQLLNQGIPVAPHTTEPMLMEYPEAITRLVTGAQRPPDPAPAPLGAPGLPNGLLSGDEDFSSIADMDFSALLSQISS

SEQ ID NO: 7 - protein, 862 aa, Artificial Sequence
  HEA4 containing two point mutations in the p65 domain that enhance transcriptional activity
MVSKLSQLQTELLAALLESGLSKEALIQALGEPGPYLLAGEGPLDKGESCGGGRGELAELPNGLGETRGSEDETDDDGEDFTPPILKELENLSPEEAAHQKAVVETLLQEDPWRVAKMVKSYLQQHNIPQREVVDTTGLNQSHLSQHLNKGTPMKTQKRAALYTWYVRKQREVAQQFTHAGQGGLIEEPTGDELPTKKGRRNRFKWGPASQQILFQAYERQKNPSKEERETLVEECNRAECIQRGVSPSQAQGLGSNLVTEVRVYNWFANRRKEEAFRHKLSAGDMRAANLWPSPLMIKRSKKNSLALSLTADQMVSALLDAEPPILYSEYDPTRPFSEASMMGLLTNLADRELVHMINWAKRVPGFVDLTLHDQVHLLECAWLEILMIGLVWRSMEHPVKLLFAPNLLLDRNQGKCVEGMVEIFDMLLATSSRFRMMNLQGEEFVCLKSIILLNSGVYTFLSSTLKSLEEKDHIHRVLDKITDTLIHLMAKAGLTLQQQHQRLAQLLLILSHIRHMSNKGMEHLYSMKCKNVVPLYDLLLEAADAHRLHAPTSRGGASVEETDQSHLATAGSTSSHSLQKYYITGEAEGFPATVEFQYLPDTDDRHRIEEKRKRTYETFQSIMKKSPFSGPTDPRPPPRRIAVPSRSSASVPKPAPQPYPFTSSLSTINYDEFPTMVFPSGQISQASALAPAPPQVLPQAPAPAPAPAMVSALAQAPAPVPVLAPGPPQAVAPPAPKPTQAGEGTLSEALLQLQFDDEDLGALLGNSTDPAVFTDLASVDNSEFQQLLNQGIPVAPHTTEPMLMEYPEAITRLVTGAQRPPDPAPAPLGAPGLPNGLLSGDEDFESIADMDFSALLSQISS

SEQ ID NO: 8 - protein, 862 aa, Artificial Sequence
  HEA3 containing three point mutations in the ER-LBD
MVSKLSQLQTELLAALLESGLSKEALIQALGEPGPYLLAGEGPLDKGESCGGGRGELAELPNGLGETRGSEDETDDDGEDFTPPILKELENLSPEEAAHQKAVVETLLQEDPWRVAKMVKSYLQQHNIPQREVVDTTGLNQSHLSQHLNKGTPMKTQKRAALYTWYVRKQREVAQQFTHAGQGGLIEEPTGDELPTKKGRRNRFKWGPASQQILFQAYERQKNPSKEERETLVEECNRAECIQRGVSPSQAQGLGSNLVTEVRVYNWFANRRKEEAFRHKLSAGDMRAANLWPSPLMIKRSKKNSLALSLTADQMVSALLDAEPPILYSEYDPTRPFSEASMMGLLTNLADRELVHMINWAKRVPGFVDLTLHDQVHLLECAWMEILMIGLVWRSMEHPGKLLFAPNLLLDRNQGKCVEGGVEIFDMLLATSSRFRMMNLQGEEFVCLKSIILLNSGVYTFLSSTLKSLEEKDHIHRVLDKITDTLIHLMAKAGLTLQQQHQRLAQLLLILSHIRHMSNKRMEHLYSMKCKNVVPLYDLLLEMLDAHRLHAPTSRGGASVEETDQSHLATAGSTSSHSLQKYYITGEAEGFPATVEFQYLPDTDDRHRIEEKRKRTYETFKSIMKKSPFSGPTDPRPPPRRIAVPSRSSASVPKPAPQPYPFTSSLSTINYDEFPTMVFPSGQISQASALAPAPPQVLPQAPAPAPAPAMVSALAQAPAPVPVLAPGPPQAVAPPAPKPTQAGEGTLSEALLQLQFDDEDLGALLGNSTDPAVFTDLASVDNSEFQQLLNQGIPVAPHTTEPMLMEYPEAITRLVTGAQRPPDPAPAPLGAPGLPNGLLSGDEDFSSIADMDFSALLSQISS

SEQ ID NO: 9 - protein, 862 aa, Artificial Sequence
  CMP8-HEA3 containing one point mutation in the p65 domain
MVSKLSQLQTELLAALLESGLSKEALIQALGEPGPYLLAGEGPLDKGESCGGGRGELAELPNGLGETRGSEDETDDDGEDFTPPILKELENLSPEEAAHQKAVVETLLQEDPWRVAKMVKSYLQQHNIPQREVVDTTGLNQSHLSQHLNKGTPMKTQKRAALYTWYVRKQREVAQQFTHAGQGGLIEEPTGDELPTKKGRRNRFKWGPASQQILFQAYERQKNPSKEERETLVEECNRAECIQRGVSPSQAQGLGSNLVTEVRVYNWFANRRKEEAFRHKLSAGDMRAANLWPSPLMIKRSKKNSLALSLTADQMVSALLDAEPPILYSEYDPTRPFSEASMMGLLTNLADRELVHMINWAKRVPGFVDLTLHDQVHLLECAWMEILMIGLVWRSMEHPGKLLFAPNLLLDRNQGKCVEGGVEIFDMLLATSSRFRMMNLQGEEFVCLKSIILLNSGVYTFLSSTLKSLEEKDHIHRVLDKITDTLIHLMAKAGLTLQQQHQRLAQLLLILSHIRHMSNKRMEHLYSMKCKNVVPLYDLLLEMLDAHRLHAPTSRGGASVEETDQSHLATAGSTSSHSLQKYYITGEAEGFPATVEFQYLPDTDDRHRIEEKRKRTYETFKSIMKKSPFSGPTDPRPPPRRIAVPSRSSASVPKPAPQPYPFTSSLSTINYDEFPTMVFPSGQISQASALAPAPPQVLPQAPAPAPAPAMVSALAQAPAPVPVLAPGPPQAVAPPAPKPTQAGEGTLSEALLQLQFDDEDLGALLGNSTDPAVFTDLASVDNSEFQQLLNQGIPVAPHTTEPMLMEYPEAITRLVTGAQRPPDPAPAPLGAPGLPNGLLSGDEDFESIADMDFSALLSQISS

SEQ ID NO: 10 - protein, 862 aa, Artificial Sequence
  CMP8-HEA3 containing one point mutation in the p65 domain
MVSKLSQLQTELLAALLESGLSKEALIQALGEPGPYLLAGEGPLDKGESCGGGRGELAELPNGLGETRGSEDETDDDGEDFTPPILKELENLSPEEAAHQKAVVETLLQEDPWRVAKMVKSYLQQHNIPQREVVDTTGLNQSHLSQHLNKGTPMKTQKRAALYTWYVRKQREVAQQFTHAGQGGLIEEPTGDELPTKKGRRNRFKWGPASQQILFQAYERQKNPSKEERETLVEECNRAECIQRGVSPSQAQGLGSNLVTEVRVYNWFANRRKEEAFRHKLSAGDMRAANLWPSPLMIKRSKKNSLALSLTADQMVSALLDAEPPILYSEYDPTRPFSEASMMGLLTNLADRELVHMINWAKRVPGFVDLTLHDQVHLLECAWMEILMIGLVWRSMEHPGKLLFAPNLLLDRNQGKCVEGGVEIFDMLLATSSRFRMMNLQGEEFVCLKSIILLNSGVYTFLSSTLKSLEEKDHIHRVLDKITDTLIHLMAKAGLTLQQQHQRLAQLLLILSHIRHMSNKRMEHLYSMKCKNVVPLYDLLLEMLDAHRLHAPTSRGGASVEETDQSHLATAGSTSSHSLQKYYITGEAEGFPATVEFQYLPDTDDRHRIEEKRKRTYETFQSIMKKSPFSGPTDPRPPPRRIAVPSRSSASVPKPAPQPYPFTSSLSTINYDEFPTMVFPSGQISQASALAPAPPQVLPQAPAPAPAPAMVSALAQAPAPVPVLAPGPPQAVAPPAPKPTQAGEGTLSEALLQLQFDDEDLGALLGNSTDPAVFTDLASVDNSEFQQLLNQGIPVAPHTTEPMLMEYPEAITRLVTGAQRPPDPAPAPLGAPGLPNGLLSGDEDFSSIADMDFSALLSQISS

SEQ ID NO: 11 - protein, 862 aa, Artificial Sequence
  CMP8-HEA3 containing two point mutations in the p65 domain
MVSKLSQLQTELLAALLESGLSKEALIQALGEPGPYLLAGEGPLDKGESCGGGRGELAELPNGLGETRGSEDETDDDGEDFTPPILKELENLSPEEAAHQKAVVETLLQEDPWRVAKMVKSYLQQHNIPQREVVDTTGLNQSHLSQHLNKGTPMKTQKRAALYTWYVRKQREVAQQFTHAGQGGLIEEPTGDELPTKKGRRNRFKWGPASQQILFQAYERQKNPSKEERETLVEECNRAECIQRGVSPSQAQGLGSNLVTEVRVYNWFANRRKEEAFRHKLSAGDMRAANLWPSPLMIKRSKKNSLALSLTADQMVSALLDAEPPILYSEYDPTRPFSEASMMGLLTNLADRELVHMINWAKRVPGFVDLTLHDQVHLLECAWMEILMIGLVWRSMEHPGKLLFAPNLLLDRNQGKCVEGGVEIFDMLLATSSRFRMMNLQGEEFVCLKSIILLNSGVYTFLSSTLKSLEEKDHIHRVLDKITDTLIHLMAKAGLTLQQQHQRLAQLLLILSHIRHMSNKRMEHLYSMKCKNVVPLYDLLLEMLDAHRLHAPTSRGGASVEETDQSHLATAGSTSSHSLQKYYITGEAEGFPATVEFQYLPDTDDRHRIEEKRKRTYETFQSIMKKSPFSGPTDPRPPPRRIAVPSRSSASVPKPAPQPYPFTSSLSTINYDEFPTMVFPSGQISQASALAPAPPQVLPQAPAPAPAPAMVSALAQAPAPVPVLAPGPPQAVAPPAPKPTQAGEGTLSEALLQLQFDDEDLGALLGNSTDPAVFTDLASVDNSEFQQLLNQGIPVAPHTTEPMLMEYPEAITRLVTGAQRPPDPAPAPLGAPGLPNGLLSGDEDFESIADMDFSALLSQISS

SEQ ID NO: 12 - DNA, 2586 bp, Unknown
  variant of the wild type HEA3 transcription factor
atggtgtccaagctgtcccagctgcagacagaactgctggcagcactgctggaaagcggcctgagcaaagaggccctgattcaggcactcggcgaacctggaccttatctgctcgctggcgaaggccctctggataagggcgagagctgtggcggaggaagaggagagctggccgagctgcctaacggcctgggcgagacaagaggcagcgaggacgagacagacgacgacggcgaggacttcaccccccccatcctgaaagagctggaaaacctgagccccgaggaagccgcccaccagaaagccgtggtggagacactgctgcaggaagatccctggcgggtcgccaagatggtcaagagctacctgcagcagcacaacatcccccagcgggaggtggtggacaccaccggcctgaaccagagccacctgagccagcacctgaacaagggcacccccatgaaaacccagaagagagccgccctgtacacttggtacgtgcggaagcagagagaggtggcccagcagtttacacacgccggccagggcggcctgatcgaggaacctaccggcgacgagctgcccaccaagaagggcagacggaaccggtttaagtggggccctgcatctcagcagatcctgttccaggcctacgagcggcagaagaaccccagcaaagaggaacgggagacactggtggaagagtgcaaccgggccgagtgcatccagagaggcgtgagcccttctcaggctcagggcctcggcagcaatctggtcaccgaagtgcgggtgtacaattggttcgccaaccggcggaaagaggaagccttccggcacaagctgtctgctggcgatatgagagccgccaacctgtggcccagccccctgatgatcaagcggagcaagaagaacagcctggccctgagcctgaccgccgatcagatggtgtccgctctgctggacgccgagccccctatcctgtacagcgagtacgaccccaccagacccttcagcgaggccagcatgatgggcctgctgaccaacctggccgaccgggagctggtgcacatgatcaactgggccaagcgggtgcccggcttcgtggacctgaccctgcacgaccaggtccacctgctggaatgtgcctggctggaaatcctgatgatcggcctcgtgtggagaagcatggaacaccccggcaagctgctgttcgcccccaacctgctcctggaccggaaccagggaaagtgcgtggagggcatggtggagatcttcgacatgctgctggccacctccagccggttccggatgatgaacctgcagggcgaggaattcgtgtgcctgaagtccatcatcctgctgaacagcggcgtgtacaccttcctgtcatccaccctgaagtccctggaagagaaggaccacatccaccgggtgctggacaagatcaccgacaccctgatccacctgatggccaaggctggcctgacactccagcagcagcaccagagactggcccagctgctgctgatcctgagccacatccggcacatgagcaacaagcggatggaacacctgtacagcatgaagtgcaagaacgtggtgcccctgtacgacctgctgctcgagatgctggatgcccacagactgcacgcccctacaagcagaggcggagccagcgtggaggaaaccgaccagtctcacctggccaccgccggcagcacaagcagccacagcctgcagaagtactacatcaccggcgaggccgagggattccctgccaccgtggagttccagtacctgcccgacaccgacgaccggcaccggatcgaggaaaagcggaagcggacctacgagacattcaagagcatcatgaagaagtcccccttcagcggccccaccgatcccagacccccccctagaagaatcgccgtgcccagcagatctagcgccagcgtgcccaagcctgccccccagccctaccctttcaccagcagcctgagcaccatcaactacgacgagttccctaccatggtgttccccagcggccagatctctcaggcctctgctctggcacctgctccacctcaggtgctgcctcaggcccctgctccagccccagcccctgccatggtgtctgcactggcccaggctccagctcctgtgcctgtgctggcccctggacctcctcaggctgtggcccctcctgcccctaaacctacccaggccggggagggaacactgtctgaggccctgctgcagctccagttcgacgacgaggatctgggagcactgctgggcaatagcaccgaccccgccgtgtttaccgacctggcctccgtggacaacagcgagttccagcagctcctcaaccagggcatccctgtcgccccacacaccaccgagcccatgctgatggaataccccgaggccatcaccagactggtcacaggcgcccagaggcctccagatccagcaccagctccactgggagcccctggcctgcctaatgggctgctgtctggcgacgaggacttctccagcattgccgacatggacttcagcgccctgctgtcccagatcagcagc

SEQ ID NO: 13 - DNA, 2586 bp, Unknown
  variant of the wild type HEA3 transcription factor
atggtgtccaagctgtcccagctgcagacagaactgctggcagcactgctggaaagcggcctgagcaaagaggccctgattcaggcactcggcgaacctggaccttatctgctcgctggcgaaggccctctggataagggcgagagctgtggcggaggaagaggagagctggccgagctgcctaacggcctgggcgagacaagaggcagcgaggacgagacagacgacgacggcgaggacttcaccccccccatcctgaaagagctggaaaacctgagccccgaggaagccgcccaccagaaagccgtggtggagacactgctgcaggaagatccctggcgggtcgccaagatggtcaagagctacctgcagcagcacaacatcccccagcgggaggtggtggacaccaccggcctgaaccagagccacctgagccagcacctgaacaagggcacccccatgaaaacccagaagagagccgccctgtacacttggtacgtgcggaagcagagagaggtggcccagcagtttacacacgccggccagggcggcctgatcgaggaacctaccggcgacgagctgcccaccaagaagggcagacggaaccggtttaagtggggccctgcatctcagcagatcctgttccaggcctacgagcggcagaagaaccccagcaaagaggaacgggagacactggtggaagagtgcaaccgggccgagtgcatccagagaggcgtgagcccttctcaggctcagggcctcggcagcaatctggtcaccgaagtgcgggtgtacaattggttcgccaaccggcggaaagaggaagccttccggcacaagctgtctgctggcgatatgagagccgccaacctgtggcccagccccctgatgatcaagcggagcaagaagaacagcctggccctgagcctgaccgccgatcagatggtgtccgctctgctggacgccgagccccctatcctgtacagcgagtacgaccccaccagacccttcagcgaggccagcatgatgggcctgctgaccaacctggccgaccgggagctggtgcacatgatcaactgggccaagcgggtgcccggcttcgtggacctgaccctgcacgaccaggtccacctgctggaatgtgcctggctggaaatcctgatgatcggcctcgtgtggagaagcatggaacaccccggcaagctgctgttcgcccccaacctgctcctggaccggaaccagggaaagtgcgtggagggcatggtggagatcttcgacatgctgctggccacctccagccggttccggatgatgaacctgcagggcgaggaattcgtgtgcctgaagtccatcatcctgctgaacagcggcgtgtacaccttcctgtcatccaccctgaagtccctggaagagaaggaccacatccaccgggtgctggacaagatcaccgacaccctgatccacctgatggccaaggctggcctgacactccagcagcagcaccagagactggcccagctgctgctgatcctgagccacatccggcacatgagcaacaagcggatggaacacctgtacagcatgaagtgcaagaacgtggtgcccctgtacgacctgctgctcgagatgctggatgcccacagactgcacgcccctacaagcagaggcggagccagcgtggaggaaaccgaccagtctcacctggccaccgccggcagcacaagcagccacagcctgcagaagtactacatcaccggcgaggccgagggattccctgccaccgtggagttccagtacctgcccgacaccgacgaccggcaccggatcgaggaaaagcggaagcggacctacgagacattcaagagcatcatgaagaagtcccccttcagcggccccaccgatcccagacccccccctagaagaatcgccgtgcccagcagatctagcgccagcgtgcccaagcctgccccccagccctaccctttcaccagcagcctgagcaccatcaactacgacgagttccctaccatggtgttccccagcggccagatctctcaggcctctgctctggcacctgctccacctcaggtgctgcctcaggcccctgctccagccccagcccctgccatggtgtctgcactggcccaggctccagctcctgtgcctgtgctggcccctggacctcctcaggctgtggcccctcctgcccctaaacctacccaggccggggagggaacactgtctgaggccctgctgcagctccagttcgacgacgaggatctgggagcactgctgggcaatagcaccgaccccgccgtgtttaccgacctggcctccgtggacaacagcgagttccagcagctcctcaaccagggcatccctgtcgccccacacaccaccgagcccatgctgatggaataccccgaggccatcaccagactggtcacaggcgcccagaggcctccagatccagcaccagctccactgggagcccctggcctgcctaatgggctgctgtctggcgacgaggacttcgagagcattgccgacatggacttcagcgccctgctgtcccagatcagcagc

SEQ ID NO: 14 - DNA, 2586 bp, Unknown
  variant of the wild type HEA3 transcription factor
atggtgtccaagctgtcccagctgcagacagaactgctggcagcactgctggaaagcggcctgagcaaagaggccctgattcaggcactcggcgaacctggaccttatctgctcgctggcgaaggccctctggataagggcgagagctgtggcggaggaagaggagagctggccgagctgcctaacggcctgggcgagacaagaggcagcgaggacgagacagacgacgacggcgaggacttcaccccccccatcctgaaagagctggaaaacctgagccccgaggaagccgcccaccagaaagccgtggtggagacactgctgcaggaagatccctggcgggtcgccaagatggtcaagagctacctgcagcagcacaacatcccccagcgggaggtggtggacaccaccggcctgaaccagagccacctgagccagcacctgaacaagggcacccccatgaaaacccagaagagagccgccctgtacacttggtacgtgcggaagcagagagaggtggcccagcagtttacacacgccggccagggcggcctgatcgaggaacctaccggcgacgagctgcccaccaagaagggcagacggaaccggtttaagtggggccctgcatctcagcagatcctgttccaggcctacgagcggcagaagaaccccagcaaagaggaacgggagacactggtggaagagtgcaaccgggccgagtgcatccagagaggcgtgagcccttctcaggctcagggcctcggcagcaatctggtcaccgaagtgcgggtgtacaattggttcgccaaccggcggaaagaggaagccttccggcacaagctgtctgctggcgatatgagagccgccaacctgtggcccagccccctgatgatcaagcggagcaagaagaacagcctggccctgagcctgaccgccgatcagatggtgtccgctctgctggacgccgagccccctatcctgtacagcgagtacgaccccaccagacccttcagcgaggccagcatgatgggcctgctgaccaacctggccgaccgggagctggtgcacatgatcaactgggccaagcgggtgcccggcttcgtggacctgaccctgcacgaccaggtccacctgctggaatgtgcctggctggaaatcctgatgatcggcctcgtgtggagaagcatggaacaccccggcaagctgctgttcgcccccaacctgctcctggaccggaaccagggaaagtgcgtggagggcatggtggagatcttcgacatgctgctggccacctccagccggttccggatgatgaacctgcagggcgaggaattcgtgtgcctgaagtccatcatcctgctgaacagcggcgtgtacaccttcctgtcatccaccctgaagtccctggaagagaaggaccacatccaccgggtgctggacaagatcaccgacaccctgatccacctgatggccaaggctggcctgacactccagcagcagcaccagagactggcccagctgctgctgatcctgagccacatccggcacatgagcaacaagcggatggaacacctgtacagcatgaagtgcaagaacgtggtgcccctgtacgacctgctgctcgagatgctggatgcccacagactgcacgcccctacaagcagaggcggagccagcgtggaggaaaccgaccagtctcacctggccaccgccggcagcacaagcagccacagcctgcagaagtactacatcaccggcgaggccgagggattccctgccaccgtggagttccagtacctgcccgacaccgacgaccggcaccggatcgaggaaaagcggaagcggacctacgagacattccagagcatcatgaagaagtcccccttcagcggccccaccgatcccagacccccccctagaagaatcgccgtgcccagcagatctagcgccagcgtgcccaagcctgccccccagccctaccctttcaccagcagcctgagcaccatcaactacgacgagttccctaccatggtgttccccagcggccagatctctcaggcctctgctctggcacctgctccacctcaggtgctgcctcaggcccctgctccagccccagcccctgccatggtgtctgcactggcccaggctccagctcctgtgcctgtgctggcccctggacctcctcaggctgtggcccctcctgcccctaaacctacccaggccggggagggaacactgtctgaggccctgctgcagctccagttcgacgacgaggatctgggagcactgctgggcaatagcaccgaccccgccgtgtttaccgacctggcctccgtggacaacagcgagttccagcagctcctcaaccagggcatccctgtcgccccacacaccaccgagcccatgctgatggaataccccgaggccatcaccagactggtcacaggcgcccagaggcctccagatccagcaccagctccactgggagcccctggcctgcctaatgggctgctgtctggcgacgaggacttctccagcattgccgacatggacttcagcgccctgctgtcccagatcagcagc

SEQ ID NO: 15 - DNA, 2586 bp, Unknown
  variant of the wild type HEA4 transcription factor
atggtgtccaagctgtcccagctgcagacagaactgctggcagcactgctggaaagcggcctgagcaaagaggccctgattcaggcactcggcgaacctggaccttatctgctcgctggcgaaggccctctggataagggcgagagctgtggcggaggaagaggagagctggccgagctgcctaacggcctgggcgagacaagaggcagcgaggacgagacagacgacgacggcgaggacttcaccccccccatcctgaaagagctggaaaacctgagccccgaggaagccgcccaccagaaagccgtggtggagacactgctgcaggaagatccctggcgggtcgccaagatggtcaagagctacctgcagcagcacaacatcccccagcgggaggtggtggacaccaccggcctgaaccagagccacctgagccagcacctgaacaagggcacccccatgaaaacccagaagagagccgccctgtacacttggtacgtgcggaagcagagagaggtggcccagcagtttacacacgccggccagggcggcctgatcgaggaacctaccggcgacgagctgcccaccaagaagggcagacggaaccggtttaagtggggccctgcatctcagcagatcctgttccaggcctacgagcggcagaagaaccccagcaaagaggaacgggagacactggtggaagagtgcaaccgggccgagtgcatccagagaggcgtgagcccttctcaggctcagggcctcggcagcaatctggtcaccgaagtgcgggtgtacaattggttcgccaaccggcggaaagaggaagccttccggcacaagctgtctgctggcgatatgagagccgccaacctgtggcccagccccctgatgatcaagcggagcaagaagaacagcctggccctgagcctgaccgccgatcagatggtgtccgctctgctggacgccgagccccctatcctgtacagcgagtacgaccccaccagacccttcagcgaggccagcatgatgggcctgctgaccaacctggccgaccgggagctggtgcacatgatcaactgggccaagcgggtgcccggcttcgtggacctgaccctgcacgaccaggtccacctgctggaatgtgcctggctggaaatcctgatgatcggcctcgtgtggagaagcatggaacaccccgtgaagctgctgttcgcccccaacctgctcctggaccggaaccagggaaagtgcgtggagggcatggtggagatcttcgacatgctgctggccacctccagccggttccggatgatgaacctgcagggcgaggaattcgtgtgcctgaagtccatcatcctgctgaacagcggcgtgtacaccttcctgtcatccaccctgaagtccctggaagagaaggaccacatccaccgggtgctggacaagatcaccgacaccctgatccacctgatggccaaggctggcctgacactccagcagcagcaccagagactggcccagctgctgctgatcctgagccacatccggcacatgagcaacaagggaatggaacacctgtacagcatgaagtgcaagaacgtggtgcccctgtacgacctgctgctcgaggctgccgatgcccacagactgcacgcccctacaagcagaggcggagccagcgtggaggaaaccgaccagtctcacctggccaccgccggcagcacaagcagccacagcctgcagaagtactacatcaccggcgaggccgagggattccctgccaccgtggagttccagtacctgcccgacaccgacgaccggcaccggatcgaggaaaagcggaagcggacctacgagacattcaagagcatcatgaagaagtcccccttcagcggccccaccgatcccagacccccccctagaagaatcgccgtgcccagcagatctagcgccagcgtgcccaagcctgccccccagccctaccctttcaccagcagcctgagcaccatcaactacgacgagttccctaccatggtgttccccagcggccagatctctcaggcctctgctctggcacctgctccacctcaggtgctgcctcaggcccctgctccagccccagcccctgccatggtgtctgcactggcccaggctccagctcctgtgcctgtgctggcccctggacctcctcaggctgtggcccctcctgcccctaaacctacccaggccggggagggaacactgtctgaggccctgctgcagctccagttcgacgacgaggatctgggagcactgctgggcaatagcaccgaccccgccgtgtttaccgacctggcctccgtggacaacagcgagttccagcagctcctcaaccagggcatccctgtcgccccacacaccaccgagcccatgctgatggaataccccgaggccatcaccagactggtcacaggcgcccagaggcctccagatccagcaccagctccactgggagcccctggcctgcctaatgggctgctgtctggcgacgaggacttctccagcattgccgacatggacttcagcgccctgctgtcccagatcagcagc

SEQ ID NO: 16 - DNA, 2586 bp, Unknown
  variant of the wild type HEA4 transcription factor
atggtgtccaagctgtcccagctgcagacagaactgctggcagcactgctggaaagcggcctgagcaaagaggccctgattcaggcactcggcgaacctggaccttatctgctcgctggcgaaggccctctggataagggcgagagctgtggcggaggaagaggagagctggccgagctgcctaacggcctgggcgagacaagaggcagcgaggacgagacagacgacgacggcgaggacttcaccccccccatcctgaaagagctggaaaacctgagccccgaggaagccgcccaccagaaagccgtggtggagacactgctgcaggaagatccctggcgggtcgccaagatggtcaagagctacctgcagcagcacaacatcccccagcgggaggtggtggacaccaccggcctgaaccagagccacctgagccagcacctgaacaagggcacccccatgaaaacccagaagagagccgccctgtacacttggtacgtgcggaagcagagagaggtggcccagcagtttacacacgccggccagggcggcctgatcgaggaacctaccggcgacgagctgcccaccaagaagggcagacggaaccggtttaagtggggccctgcatctcagcagatcctgttccaggcctacgagcggcagaagaaccccagcaaagaggaacgggagacactggtggaagagtgcaaccgggccgagtgcatccagagaggcgtgagcccttctcaggctcagggcctcggcagcaatctggtcaccgaagtgcgggtgtacaattggttcgccaaccggcggaaagaggaagccttccggcacaagctgtctgctggcgatatgagagccgccaacctgtggcccagccccctgatgatcaagcggagcaagaagaacagcctggccctgagcctgaccgccgatcagatggtgtccgctctgctggacgccgagccccctatcctgtacagcgagtacgaccccaccagacccttcagcgaggccagcatgatgggcctgctgaccaacctggccgaccgggagctggtgcacatgatcaactgggccaagcgggtgcccggcttcgtggacctgaccctgcacgaccaggtccacctgctggaatgtgcctggctggaaatcctgatgatcggcctcgtgtggagaagcatggaacaccccgtgaagctgctgttcgcccccaacctgctcctggaccggaaccagggaaagtgcgtggagggcatggtggagatcttcgacatgctgctggccacctccagccggttccggatgatgaacctgcagggcgaggaattcgtgtgcctgaagtccatcatcctgctgaacagcggcgtgtacaccttcctgtcatccaccctgaagtccctggaagagaaggaccacatccaccgggtgctggacaagatcaccgacaccctgatccacctgatggccaaggctggcctgacactccagcagcagcaccagagactggcccagctgctgctgatcctgagccacatccggcacatgagcaacaagggaatggaacacctgtacagcatgaagtgcaagaacgtggtgcccctgtacgacctgctgctcgaggctgccgatgcccacagactgcacgcccctacaagcagaggcggagccagcgtggaggaaaccgaccagtctcacctggccaccgccggcagcacaagcagccacagcctgcagaagtactacatcaccggcgaggccgagggattccctgccaccgtggagttccagtacctgcccgacaccgacgaccggcaccggatcgaggaaaagcggaagcggacctacgagacattcaagagcatcatgaagaagtcccccttcagcggccccaccgatcccagacccccccctagaagaatcgccgtgcccagcagatctagcgccagcgtgcccaagcctgccccccagccctaccctttcaccagcagcctgagcaccatcaactacgacgagttccctaccatggtgttccccagcggccagatctctcaggcctctgctctggcacctgctccacctcaggtgctgcctcaggcccctgctccagccccagcccctgccatggtgtctgcactggcccaggctccagctcctgtgcctgtgctggcccctggacctcctcaggctgtggcccctcctgcccctaaacctacccaggccggggagggaacactgtctgaggccctgctgcagctccagttcgacgacgaggatctgggagcactgctgggcaatagcaccgaccccgccgtgtttaccgacctggcctccgtggacaacagcgagttccagcagctcctcaaccagggcatccctgtcgccccacacaccaccgagcccatgctgatggaataccccgaggccatcaccagactggtcacaggcgcccagaggcctccagatccagcaccagctccactgggagcccctggcctgcctaatgggctgctgtctggcgacgaggacttcgagagcattgccgacatggacttcagcgccctgctgtcccagatcagcagc

SEQ ID NO: 17 - DNA, 2586 bp, Unknown
  variant of the wild type HEA4 transcription factor
atggtgtccaagctgtcccagctgcagacagaactgctggcagcactgctggaaagcggcctgagcaaagaggccctgattcaggcactcggcgaacctggaccttatctgctcgctggcgaaggccctctggataagggcgagagctgtggcggaggaagaggagagctggccgagctgcctaacggcctgggcgagacaagaggcagcgaggacgagacagacgacgacggcgaggacttcaccccccccatcctgaaagagctggaaaacctgagccccgaggaagccgcccaccagaaagccgtggtggagacactgctgcaggaagatccctggcgggtcgccaagatggtcaagagctacctgcagcagcacaacatcccccagcgggaggtggtggacaccaccggcctgaaccagagccacctgagccagcacctgaacaagggcacccccatgaaaacccagaagagagccgccctgtacacttggtacgtgcggaagcagagagaggtggcccagcagtttacacacgccggccagggcggcctgatcgaggaacctaccggcgacgagctgcccaccaagaagggcagacggaaccggtttaagtggggccctgcatctcagcagatcctgttccaggcctacgagcggcagaagaaccccagcaaagaggaacgggagacactggtggaagagtgcaaccgggccgagtgcatccagagaggcgtgagcccttctcaggctcagggcctcggcagcaatctggtcaccgaagtgcgggtgtacaattggttcgccaaccggcggaaagaggaagccttccggcacaagctgtctgctggcgatatgagagccgccaacctgtggcccagccccctgatgatcaagcggagcaagaagaacagcctggccctgagcctgaccgccgatcagatggtgtccgctctgctggacgccgagccccctatcctgtacagcgagtacgaccccaccagacccttcagcgaggccagcatgatgggcctgctgaccaacctggccgaccgggagctggtgcacatgatcaactgggccaagcgggtgcccggcttcgtggacctgaccctgcacgaccaggtccacctgctggaatgtgcctggctggaaatcctgatgatcggcctcgtgtggagaagcatggaacaccccgtgaagctgctgttcgcccccaacctgctcctggaccggaaccagggaaagtgcgtggagggcatggtggagatcttcgacatgctgctggccacctccagccggttccggatgatgaacctgcagggcgaggaattcgtgtgcctgaagtccatcatcctgctgaacagcggcgtgtacaccttcctgtcatccaccctgaagtccctggaagagaaggaccacatccaccgggtgctggacaagatcaccgacaccctgatccacctgatggccaaggctggcctgacactccagcagcagcaccagagactggcccagctgctgctgatcctgagccacatccggcacatgagcaacaagggaatggaacacctgtacagcatgaagtgcaagaacgtggtgcccctgtacgacctgctgctcgaggctgccgatgcccacagactgcacgcccctacaagcagaggcggagccagcgtggaggaaaccgaccagtctcacctggccaccgccggcagcacaagcagccacagcctgcagaagtactacatcaccggcgaggccgagggattccctgccaccgtggagttccagtacctgcccgacaccgacgaccggcaccggatcgaggaaaagcggaagcggacctacgagacattccagagcatcatgaagaagtcccccttcagcggccccaccgatcccagacccccccctagaagaatcgccgtgcccagcagatctagcgccagcgtgcccaagcctgccccccagccctaccctttcaccagcagcctgagcaccatcaactacgacgagttccctaccatggtgttccccagcggccagatctctcaggcctctgctctggcacctgctccacctcaggtgctgcctcaggcccctgctccagccccagcccctgccatggtgtctgcactggcccaggctccagctcctgtgcctgtgctggcccctggacctcctcaggctgtggcccctcctgcccctaaacctacccaggccggggagggaacactgtctgaggccctgctgcagctccagttcgacgacgaggatctgggagcactgctgggcaatagcaccgaccccgccgtgtttaccgacctggcctccgtggacaacagcgagttccagcagctcctcaaccagggcatccctgtcgccccacacaccaccgagcccatgctgatggaataccccgaggccatcaccagactggtcacaggcgcccagaggcctccagatccagcaccagctccactgggagcccctggcctgcctaatgggctgctgtctggcgacgaggacttctccagcattgccgacatggacttcagcgccctgctgtcccagatcagcagc

SEQ ID NO: 18 - DNA, 2586 bp, Unknown
  variant of the wild type HEA4 transcription factor
atggtgtccaagctgtcccagctgcagacagaactgctggcagcactgctggaaagcggcctgagcaaagaggccctgattcaggcactcggcgaacctggaccttatctgctcgctggcgaaggccctctggataagggcgagagctgtggcggaggaagaggagagctggccgagctgcctaacggcctgggcgagacaagaggcagcgaggacgagacagacgacgacggcgaggacttcaccccccccatcctgaaagagctggaaaacctgagccccgaggaagccgcccaccagaaagccgtggtggagacactgctgcaggaagatccctggcgggtcgccaagatggtcaagagctacctgcagcagcacaacatcccccagcgggaggtggtggacaccaccggcctgaaccagagccacctgagccagcacctgaacaagggcacccccatgaaaacccagaagagagccgccctgtacacttggtacgtgcggaagcagagagaggtggcccagcagtttacacacgccggccagggcggcctgatcgaggaacctaccggcgacgagctgcccaccaagaagggcagacggaaccggtttaagtggggccctgcatctcagcagatcctgttccaggcctacgagcggcagaagaaccccagcaaagaggaacgggagacactggtggaagagtgcaaccgggccgagtgcatccagagaggcgtgagcccttctcaggctcagggcctcggcagcaatctggtcaccgaagtgcgggtgtacaattggttcgccaaccggcggaaagaggaagccttccggcacaagctgtctgctggcgatatgagagccgccaacctgtggcccagccccctgatgatcaagcggagcaagaagaacagcctggccctgagcctgaccgccgatcagatggtgtccgctctgctggacgccgagccccctatcctgtacagcgagtacgaccccaccagacccttcagcgaggccagcatgatgggcctgctgaccaacctggccgaccgggagctggtgcacatgatcaactgggccaagcgggtgcccggcttcgtggacctgaccctgcacgaccaggtccacctgctggaatgtgcctggctggaaatcctgatgatcggcctcgtgtggagaagcatggaacaccccgtgaagctgctgttcgcccccaacctgctcctggaccggaaccagggaaagtgcgtggagggcatggtggagatcttcgacatgctgctggccacctccagccggttccggatgatgaacctgcagggcgaggaattcgtgtgcctgaagtccatcatcctgctgaacagcggcgtgtacaccttcctgtcatccaccctgaagtccctggaagagaaggaccacatccaccgggtgctggacaagatcaccgacaccctgatccacctgatggccaaggctggcctgacactccagcagcagcaccagagactggcccagctgctgctgatcctgagccacatccggcacatgagcaacaagggaatggaacacctgtacagcatgaagtgcaagaacgtggtgcccctgtacgacctgctgctcgaggctgccgatgcccacagactgcacgcccctacaagcagaggcggagccagcgtggaggaaaccgaccagtctcacctggccaccgccggcagcacaagcagccacagcctgcagaagtactacatcaccggcgaggccgagggattccctgccaccgtggagttccagtacctgcccgacaccgacgaccggcaccggatcgaggaaaagcggaagcggacctacgagacattccagagcatcatgaagaagtcccccttcagcggccccaccgatcccagacccccccctagaagaatcgccgtgcccagcagatctagcgccagcgtgcccaagcctgccccccagccctaccctttcaccagcagcctgagcaccatcaactacgacgagttccctaccatggtgttccccagcggccagatctctcaggcctctgctctggcacctgctccacctcaggtgctgcctcaggcccctgctccagccccagcccctgccatggtgtctgcactggcccaggctccagctcctgtgcctgtgctggcccctggacctcctcaggctgtggcccctcctgcccctaaacctacccaggccggggagggaacactgtctgaggccctgctgcagctccagttcgacgacgaggatctgggagcactgctgggcaatagcaccgaccccgccgtgtttaccgacctggcctccgtggacaacagcgagttccagcagctcctcaaccagggcatccctgtcgccccacacaccaccgagcccatgctgatggaataccccgaggccatcaccagactggtcacaggcgcccagaggcctccagatccagcaccagctccactgggagcccctggcctgcctaatgggctgctgtctggcgacgaggacttcgagagcattgccgacatggacttcagcgccctgctgtcccagatcagcagc

SEQ ID NO: 19 - DNA, 2586 bp, Unknown
  variant of the wild type HEA3 transcription factor
atggtgtccaagctgtcccagctgcagacagaactgctggcagcactgctggaaagcggcctgagcaaagaggccctgattcaggcactcggcgaacctggaccttatctgctcgctggcgaaggccctctggataagggcgagagctgtggcggaggaagaggagagctggccgagctgcctaacggcctgggcgagacaagaggcagcgaggacgagacagacgacgacggcgaggacttcaccccccccatcctgaaagagctggaaaacctgagccccgaggaagccgcccaccagaaagccgtggtggagacactgctgcaggaagatccctggcgggtcgccaagatggtcaagagctacctgcagcagcacaacatcccccagcgggaggtggtggacaccaccggcctgaaccagagccacctgagccagcacctgaacaagggcacccccatgaaaacccagaagagagccgccctgtacacttggtacgtgcggaagcagagagaggtggcccagcagtttacacacgccggccagggcggcctgatcgaggaacctaccggcgacgagctgcccaccaagaagggcagacggaaccggtttaagtggggccctgcatctcagcagatcctgttccaggcctacgagcggcagaagaaccccagcaaagaggaacgggagacactggtggaagagtgcaaccgggccgagtgcatccagagaggcgtgagcccttctcaggctcagggcctcggcagcaatctggtcaccgaagtgcgggtgtacaattggttcgccaaccggcggaaagaggaagccttccggcacaagctgtctgctggcgatatgagagccgccaacctgtggcccagccccctgatgatcaagcggagcaagaagaacagcctggccctgagcctgaccgccgatcagatggtgtccgctctgctggacgccgagccccctatcctgtacagcgagtacgaccccaccagacccttcagcgaggccagcatgatgggcctgctgaccaacctggccgaccgggagctggtgcacatgatcaactgggccaagcgggtgcccggcttcgtggacctgaccctgcacgaccaggtccacctgctggaatgtgcctggatggaaatcctgatgatcggcctcgtgtggagaagcatggaacaccccggcaagctgctgttcgcccccaacctgctcctggaccggaaccagggaaagtgcgtggagggcggcgtggagatcttcgacatgctgctggccacctccagccggttccggatgatgaacctgcagggcgaggaattcgtgtgcctgaagtccatcatcctgctgaacagcggcgtgtacaccttcctgtcatccaccctgaagtccctggaagagaaggaccacatccaccgggtgctggacaagatcaccgacaccctgatccacctgatggccaaggctggcctgacactccagcagcagcaccagagactggcccagctgctgctgatcctgagccacatccggcacatgagcaacaagcggatggaacacctgtacagcatgaagtgcaagaacgtggtgcccctgtacgacctgctgctcgagatgctggatgcccacagactgcacgcccctacaagcagaggcggagccagcgtggaggaaaccgaccagtctcacctggccaccgccggcagcacaagcagccacagcctgcagaagtactacatcaccggcgaggccgagggattccctgccaccgtggagttccagtacctgcccgacaccgacgaccggcaccggatcgaggaaaagcggaagcggacctacgagacattcaagagcatcatgaagaagtcccccttcagcggccccaccgatcccagacccccccctagaagaatcgccgtgcccagcagatctagcgccagcgtgcccaagcctgccccccagccctaccctttcaccagcagcctgagcaccatcaactacgacgagttccctaccatggtgttccccagcggccagatctctcaggcctctgctctggcacctgctccacctcaggtgctgcctcaggcccctgctccagccccagcccctgccatggtgtctgcactggcccaggctccagctcctgtgcctgtgctggcccctggacctcctcaggctgtggcccctcctgcccctaaacctacccaggccggggagggaacactgtctgaggccctgctgcagctccagttcgacgacgaggatctgggagcactgctgggcaatagcaccgaccccgccgtgtttaccgacctggcctccgtggacaacagcgagttccagcagctcctcaaccagggcatccctgtcgccccacacaccaccgagcccatgctgatggaataccccgaggccatcaccagactggtcacaggcgcccagaggcctccagatccagcaccagctccactgggagcccctggcctgcctaatgggctgctgtctggcgacgaggacttctccagcattgccgacatggacttcagcgccctgctgtcccagatcagcagc

SEQ ID NO: 20 - DNA, 2586 bp, Unknown
  variant of the wild type HEA3 transcription factor
atggtgtccaagctgtcccagctgcagacagaactgctggcagcactgctggaaagcggcctgagcaaagaggccctgattcaggcactcggcgaacctggaccttatctgctcgctggcgaaggccctctggataagggcgagagctgtggcggaggaagaggagagctggccgagctgcctaacggcctgggcgagacaagaggcagcgaggacgagacagacgacgacggcgaggacttcaccccccccatcctgaaagagctggaaaacctgagccccgaggaagccgcccaccagaaagccgtggtggagacactgctgcaggaagatccctggcgggtcgccaagatggtcaagagctacctgcagcagcacaacatcccccagcgggaggtggtggacaccaccggcctgaaccagagccacctgagccagcacctgaacaagggcacccccatgaaaacccagaagagagccgccctgtacacttggtacgtgcggaagcagagagaggtggcccagcagtttacacacgccggccagggcggcctgatcgaggaacctaccggcgacgagctgcccaccaagaagggcagacggaaccggtttaagtggggccctgcatctcagcagatcctgttccaggcctacgagcggcagaagaaccccagcaaagaggaacgggagacactggtggaagagtgcaaccgggccgagtgcatccagagaggcgtgagcccttctcaggctcagggcctcggcagcaatctggtcaccgaagtgcgggtgtacaattggttcgccaaccggcggaaagaggaagccttccggcacaagctgtctgctggcgatatgagagccgccaacctgtggcccagccccctgatgatcaagcggagcaagaagaacagcctggccctgagcctgaccgccgatcagatggtgtccgctctgctggacgccgagccccctatcctgtacagcgagtacgaccccaccagacccttcagcgaggccagcatgatgggcctgctgaccaacctggccgaccgggagctggtgcacatgatcaactgggccaagcgggtgcccggcttcgtggacctgaccctgcacgaccaggtccacctgctggaatgtgcctggatggaaatcctgatgatcggcctcgtgtggagaagcatggaacaccccggcaagctgctgttcgcccccaacctgctcctggaccggaaccagggaaagtgcgtggagggcggcgtggagatcttcgacatgctgctggccacctccagccggttccggatgatgaacctgcagggcgaggaattcgtgtgcctgaagtccatcatcctgctgaacagcggcgtgtacaccttcctgtcatccaccctgaagtccctggaagagaaggaccacatccaccgggtgctggacaagatcaccgacaccctgatccacctgatggccaaggctggcctgacactccagcagcagcaccagagactggcccagctgctgctgatcctgagccacatccggcacatgagcaacaagcggatggaacacctgtacagcatgaagtgcaagaacgtggtgcccctgtacgacctgctgctcgagatgctggatgcccacagactgcacgcccctacaagcagaggcggagccagcgtggaggaaaccgaccagtctcacctggccaccgccggcagcacaagcagccacagcctgcagaagtactacatcaccggcgaggccgagggattccctgccaccgtggagttccagtacctgcccgacaccgacgaccggcaccggatcgaggaaaagcggaagcggacctacgagacattcaagagcatcatgaagaagtcccccttcagcggccccaccgatcccagacccccccctagaagaatcgccgtgcccagcagatctagcgccagcgtgcccaagcctgccccccagccctaccctttcaccagcagcctgagcaccatcaactacgacgagttccctaccatggtgttccccagcggccagatctctcaggcctctgctctggcacctgctccacctcaggtgctgcctcaggcccctgctccagccccagcccctgccatggtgtctgcactggcccaggctccagctcctgtgcctgtgctggcccctggacctcctcaggctgtggcccctcctgcccctaaacctacccaggccggggagggaacactgtctgaggccctgctgcagctccagttcgacgacgaggatctgggagcactgctgggcaatagcaccgaccccgccgtgtttaccgacctggcctccgtggacaacagcgagttccagcagctcctcaaccagggcatccctgtcgccccacacaccaccgagcccatgctgatggaataccccgaggccatcaccagactggtcacaggcgcccagaggcctccagatccagcaccagctccactgggagcccctggcctgcctaatgggctgctgtctggcgacgaggacttcgagagcattgccgacatggacttcagcgccctgctgtcccagatcagcagc

SEQ ID NO: 21 - DNA, 2586 bp, Unknown
  variant of the wild type HEA3 transcription factor
atggtgtccaagctgtcccagctgcagacagaactgctggcagcactgctggaaagcggcctgagcaaagaggccctgattcaggcactcggcgaacctggaccttatctgctcgctggcgaaggccctctggataagggcgagagctgtggcggaggaagaggagagctggccgagctgcctaacggcctgggcgagacaagaggcagcgaggacgagacagacgacgacggcgaggacttcaccccccccatcctgaaagagctggaaaacctgagccccgaggaagccgcccaccagaaagccgtggtggagacactgctgcaggaagatccctggcgggtcgccaagatggtcaagagctacctgcagcagcacaacatcccccagcgggaggtggtggacaccaccggcctgaaccagagccacctgagccagcacctgaacaagggcacccccatgaaaacccagaagagagccgccctgtacacttggtacgtgcggaagcagagagaggtggcccagcagtttacacacgccggccagggcggcctgatcgaggaacctaccggcgacgagctgcccaccaagaagggcagacggaaccggtttaagtggggccctgcatctcagcagatcctgttccaggcctacgagcggcagaagaaccccagcaaagaggaacgggagacactggtggaagagtgcaaccgggccgagtgcatccagagaggcgtgagcccttctcaggctcagggcctcggcagcaatctggtcaccgaagtgcgggtgtacaattggttcgccaaccggcggaaagaggaagccttccggcacaagctgtctgctggcgatatgagagccgccaacctgtggcccagccccctgatgatcaagcggagcaagaagaacagcctggccctgagcctgaccgccgatcagatggtgtccgctctgctggacgccgagccccctatcctgtacagcgagtacgaccccaccagacccttcagcgaggccagcatgatgggcctgctgaccaacctggccgaccgggagctggtgcacatgatcaactgggccaagcgggtgcccggcttcgtggacctgaccctgcacgaccaggtccacctgctggaatgtgcctggatggaaatcctgatgatcggcctcgtgtggagaagcatggaacaccccggcaagctgctgttcgcccccaacctgctcctggaccggaaccagggaaagtgcgtggagggcggcgtggagatcttcgacatgctgctggccacctccagccggttccggatgatgaacctgcagggcgaggaattcgtgtgcctgaagtccatcatcctgctgaacagcggcgtgtacaccttcctgtcatccaccctgaagtccctggaagagaaggaccacatccaccgggtgctggacaagatcaccgacaccctgatccacctgatggccaaggctggcctgacactccagcagcagcaccagagactggcccagctgctgctgatcctgagccacatccggcacatgagcaacaagcggatggaacacctgtacagcatgaagtgcaagaacgtggtgcccctgtacgacctgctgctcgagatgctggatgcccacagactgcacgcccctacaagcagaggcggagccagcgtggaggaaaccgaccagtctcacctggccaccgccggcagcacaagcagccacagcctgcagaagtactacatcaccggcgaggccgagggattccctgccaccgtggagttccagtacctgcccgacaccgacgaccggcaccggatcgaggaaaagcggaagcggacctacgagacattccagagcatcatgaagaagtcccccttcagcggccccaccgatcccagacccccccctagaagaatcgccgtgcccagcagatctagcgccagcgtgcccaagcctgccccccagccctaccctttcaccagcagcctgagcaccatcaactacgacgagttccctaccatggtgttccccagcggccagatctctcaggcctctgctctggcacctgctccacctcaggtgctgcctcaggcccctgctccagccccagcccctgccatggtgtctgcactggcccaggctccagctcctgtgcctgtgctggcccctggacctcctcaggctgtggcccctcctgcccctaaacctacccaggccggggagggaacactgtctgaggccctgctgcagctccagttcgacgacgaggatctgggagcactgctgggcaatagcaccgaccccgccgtgtttaccgacctggcctccgtggacaacagcgagttccagcagctcctcaaccagggcatccctgtcgccccacacaccaccgagcccatgctgatggaataccccgaggccatcaccagactggtcacaggcgcccagaggcctccagatccagcaccagctccactgggagcccctggcctgcctaatgggctgctgtctggcgacgaggacttctccagcattgccgacatggacttcagcgccctgctgtcccagatcagcagc

SEQ ID NO: 22 - DNA, 2586 bp, Unknown
  variant of the wild type HEA3 transcription factor
atggtgtccaagctgtcccagctgcagacagaactgctggcagcactgctggaaagcggcctgagcaaagaggccctgattcaggcactcggcgaacctggaccttatctgctcgctggcgaaggccctctggataagggcgagagctgtggcggaggaagaggagagctggccgagctgcctaacggcctgggcgagacaagaggcagcgaggacgagacagacgacgacggcgaggacttcaccccccccatcctgaaagagctggaaaacctgagccccgaggaagccgcccaccagaaagccgtggtggagacactgctgcaggaagatccctggcgggtcgccaagatggtcaagagctacctgcagcagcacaacatcccccagcgggaggtggtggacaccaccggcctgaaccagagccacctgagccagcacctgaacaagggcacccccatgaaaacccagaagagagccgccctgtacacttggtacgtgcggaagcagagagaggtggcccagcagtttacacacgccggccagggcggcctgatcgaggaacctaccggcgacgagctgcccaccaagaagggcagacggaaccggtttaagtggggccctgcatctcagcagatcctgttccaggcctacgagcggcagaagaaccccagcaaagaggaacgggagacactggtggaagagtgcaaccgggccgagtgcatccagagaggcgtgagcccttctcaggctcagggcctcggcagcaatctggtcaccgaagtgcgggtgtacaattggttcgccaaccggcggaaagaggaagccttccggcacaagctgtctgctggcgatatgagagccgccaacctgtggcccagccccctgatgatcaagcggagcaagaagaacagcctggccctgagcctgaccgccgatcagatggtgtccgctctgctggacgccgagccccctatcctgtacagcgagtacgaccccaccagacccttcagcgaggccagcatgatgggcctgctgaccaacctggccgaccgggagctggtgcacatgatcaactgggccaagcgggtgcccggcttcgtggacctgaccctgcacgaccaggtccacctgctggaatgtgcctggatggaaatcctgatgatcggcctcgtgtggagaagcatggaacaccccggcaagctgctgttcgcccccaacctgctcctggaccggaaccagggaaagtgcgtggagggcggcgtggagatcttcgacatgctgctggccacctccagccggttccggatgatgaacctgcagggcgaggaattcgtgtgcctgaagtccatcatcctgctgaacagcggcgtgtacaccttcctgtcatccaccctgaagtccctggaagagaaggaccacatccaccgggtgctggacaagatcaccgacaccctgatccacctgatggccaaggctggcctgacactccagcagcagcaccagagactggcccagctgctgctgatcctgagccacatccggcacatgagcaacaagcggatggaacacctgtacagcatgaagtgcaagaacgtggtgcccctgtacgacctgctgctcgagatgctggatgcccacagactgcacgcccctacaagcagaggcggagccagcgtggaggaaaccgaccagtctcacctggccaccgccggcagcacaagcagccacagcctgcagaagtactacatcaccggcgaggccgagggattccctgccaccgtggagttccagtacctgcccgacaccgacgaccggcaccggatcgaggaaaagcggaagcggacctacgagacattccagagcatcatgaagaagtcccccttcagcggccccaccgatcccagacccccccctagaagaatcgccgtgcccagcagatctagcgccagcgtgcccaagcctgccccccagccctaccctttcaccagcagcctgagcaccatcaactacgacgagttccctaccatggtgttccccagcggccagatctctcaggcctctgctctggcacctgctccacctcaggtgctgcctcaggcccctgctccagccccagcccctgccatggtgtctgcactggcccaggctccagctcctgtgcctgtgctggcccctggacctcctcaggctgtggcccctcctgcccctaaacctacccaggccggggagggaacactgtctgaggccctgctgcagctccagttcgacgacgaggatctgggagcactgctgggcaatagcaccgaccccgccgtgtttaccgacctggcctccgtggacaacagcgagttccagcagctcctcaaccagggcatccctgtcgccccacacaccaccgagcccatgctgatggaataccccgaggccatcaccagactggtcacaggcgcccagaggcctccagatccagcaccagctccactgggagcccctggcctgcctaatgggctgctgtctggcgacgaggacttcgagagcattgccgacatggacttcagcgccctgctgtcccagatcagcagc

SEQ ID NO: 23 - DNA, 138 bp, Unknown
  7xHBD/mE1B promoter
tagttaataatctacaatagttaataatctacaatagttaataatctacaatagttaataatctacaatagttaataatctacaatagttaataatctacaatagttaataatctacaagagctcagggtatataatg

SEQ ID NO: 24 - DNA, 1941 bp, Unknown
  HEA4(VP64) chimeric transcription factor
atggtgtccaagctgtcccagctgcagacagaactgctggcagcactgctggaaagcggcctgagcaaagaggccctgattcaggcactcggcgaacctggaccttatctgctcgctggcgaaggccctctggataagggcgagagctgtggcggaggaagaggagagctggccgagctgcctaacggcctgggcgagacaagaggcagcgaggacgagacagacgacgacggcgaggacttcaccccccccatcctgaaagagctggaaaacctgagccccgaggaagccgcccaccagaaagccgtggtggagacactgctgcaggaagatccctggcgggtcgccaagatggtcaagagctacctgcagcagcacaacatcccccagcgggaggtggtggacaccaccggcctgaaccagagccacctgagccagcacctgaacaagggcacccccatgaaaacccagaagagagccgccctgtacacttggtacgtgcggaagcagagagaggtggcccagcagtttacacacgccggccagggcggcctgatcgaggaacctaccggcgacgagctgcccaccaagaagggcagacggaaccggtttaagtggggccctgcatctcagcagatcctgttccaggcctacgagcggcagaagaaccccagcaaagaggaacgggagacactggtggaagagtgcaaccgggccgagtgcatccagagaggcgtgagcccttctcaggctcagggcctcggcagcaatctggtcaccgaagtgcgggtgtacaattggttcgccaaccggcggaaagaggaagccttccggcacaagctgtctgctggcgatatgagagccgccaacctgtggcccagccccctgatgatcaagcggagcaagaagaacagcctggccctgagcctgaccgccgatcagatggtgtccgctctgctggacgccgagccccctatcctgtacagcgagtacgaccccaccagacccttcagcgaggccagcatgatgggcctgctgaccaacctggccgaccgggagctggtgcacatgatcaactgggccaagcgggtgcccggcttcgtggacctgaccctgcacgaccaggtccacctgctggaatgtgcctggctggaaatcctgatgatcggcctcgtgtggagaagcatggaacaccccgtgaagctgctgttcgcccccaacctgctcctggaccggaaccagggaaagtgcgtggagggcatggtggagatcttcgacatgctgctggccacctccagccggttccggatgatgaacctgcagggcgaggaattcgtgtgcctgaagtccatcatcctgctgaacagcggcgtgtacaccttcctgtcatccaccctgaagtccctggaagagaaggaccacatccaccgggtgctggacaagatcaccgacaccctgatccacctgatggccaaggctggcctgacactccagcagcagcaccagagactggcccagctgctgctgatcctgagccacatccggcacatgagcaacaagggaatggaacacctgtacagcatgaagtgcaagaacgtggtgcccctgtacgacctgctgctcgaggctgccgatgcccacagactgcacgcccctacaagcagaggcggagccagcgtggaggaaaccgaccagtctcacctggccaccgccggcagcacaagcagccacagcctgcagaagtactacatcaccggcgaggccgagggattccctgccaccgtggacgctctggacgacttcgaccttgacatgttgggttccgacgcgctggatgattttgatttggacatgctgggaagcgacgcactggatgactttgatctcgatatgctcggctctgacgcattggacgacttcgacttggatatgctgggttct

SEQ ID NO: 25 - protein, 647 aa, Artificial Sequence
  HEA4(VP64) chimeric transcription factor
MVSKLSQLQTELLAALLESGLSKEALIQALGEPGPYLLAGEGPLDKGESCGGGRGELAELPNGLGETRGSEDETDDDGEDFTPPILKELENLSPEEAAHQKAVVETLLQEDPWRVAKMVKSYLQQHNIPQREVVDTTGLNQSHLSQHLNKGTPMKTQKRAALYTWYVRKQREVAQQFTHAGQGGLIEEPTGDELPTKKGRRNRFKWGPASQQILFQAYERQKNPSKEERETLVEECNRAECIQRGVSPSQAQGLGSNLVTEVRVYNWFANRRKEEAFRHKLSAGDMRAANLWPSPLMIKRSKKNSLALSLTADQMVSALLDAEPPILYSEYDPTRPFSEASMMGLLTNLADRELVHMINWAKRVPGFVDLTLHDQVHLLECAWLEILMIGLVWRSMEHPVKLLFAPNLLLDRNQGKCVEGMVEIFDMLLATSSRFRMMNLQGEEFVCLKSIILLNSGVYTFLSSTLKSLEEKDHIHRVLDKITDTLIHLMAKAGLTLQQQHQRLAQLLLILSHIRHMSNKGMEHLYSMKCKNVVPLYDLLLEAADAHRLHAPTSRGGASVEETDQSHLATAGSTSSHSLQKYYITGEAEGFPATVDALDDFDLDMLGSDALDDFDLDMLGSDALDDFDLDMLGSDALDDFDLDMLGS

SEQ ID NO: 26 - DNA, 2262 bp, Unknown
  HEA4(HSF-1) chimeric transcription factor
atggtgtccaagctgtcccagctgcagacagaactgctggcagcactgctggaaagcggcctgagcaaagaggccctgattcaggcactcggcgaacctggaccttatctgctcgctggcgaaggccctctggataagggcgagagctgtggcggaggaagaggagagctggccgagctgcctaacggcctgggcgagacaagaggcagcgaggacgagacagacgacgacggcgaggacttcaccccccccatcctgaaagagctggaaaacctgagccccgaggaagccgcccaccagaaagccgtggtggagacactgctgcaggaagatccctggcgggtcgccaagatggtcaagagctacctgcagcagcacaacatcccccagcgggaggtggtggacaccaccggcctgaaccagagccacctgagccagcacctgaacaagggcacccccatgaaaacccagaagagagccgccctgtacacttggtacgtgcggaagcagagagaggtggcccagcagtttacacacgccggccagggcggcctgatcgaggaacctaccggcgacgagctgcccaccaagaagggcagacggaaccggtttaagtggggccctgcatctcagcagatcctgttccaggcctacgagcggcagaagaaccccagcaaagaggaacgggagacactggtggaagagtgcaaccgggccgagtgcatccagagaggcgtgagcccttctcaggctcagggcctcggcagcaatctggtcaccgaagtgcgggtgtacaattggttcgccaaccggcggaaagaggaagccttccggcacaagctgtctgctggcgatatgagagccgccaacctgtggcccagccccctgatgatcaagcggagcaagaagaacagcctggccctgagcctgaccgccgatcagatggtgtccgctctgctggacgccgagccccctatcctgtacagcgagtacgaccccaccagacccttcagcgaggccagcatgatgggcctgctgaccaacctggccgaccgggagctggtgcacatgatcaactgggccaagcgggtgcccggcttcgtggacctgaccctgcacgaccaggtccacctgctggaatgtgcctggctggaaatcctgatgatcggcctcgtgtggagaagcatggaacaccccgtgaagctgctgttcgcccccaacctgctcctggaccggaaccagggaaagtgcgtggagggcatggtggagatcttcgacatgctgctggccacctccagccggttccggatgatgaacctgcagggcgaggaattcgtgtgcctgaagtccatcatcctgctgaacagcggcgtgtacaccttcctgtcatccaccctgaagtccctggaagagaaggaccacatccaccgggtgctggacaagatcaccgacaccctgatccacctgatggccaaggctggcctgacactccagcagcagcaccagagactggcccagctgctgctgatcctgagccacatccggcacatgagcaacaagggaatggaacacctgtacagcatgaagtgcaagaacgtggtgcccctgtacgacctgctgctcgaggctgccgatgcccacagactgcacgcccctacaagcagaggcggagccagcgtggaggaaaccgaccagtctcacctggccaccgccggcagcacaagcagccacagcctgcagaagtactacatcaccggcgaggccgagggattccctgccaccgtggaaaagtgcctcagcgtagcctgcctggacaagaatgagctcagtgaccacttggatgctatggactccaacctggataacctgcagaccatgctgagcagccacggcttcagcgtggacaccagtgccctgctggacctgttcagcccctcggtgaccgtgcccgacatgagcctgcctgaccttgacagcagcctggccagtatccaagagctcctgtctccccaggagccccccaggcctcccgaggcagagaacagcagcccggattcagggaagcagctggtgcactacacagcgcagccgctgttcctgctggaccccggctccgtggacaccgggagcaacgacctgccggtgctgtttgagctgggagagggctcctacttctccgaaggggacggcttcgccgaggaccccaccatctccctgctgacaggctcggagcctcccaaagccaaggaccccactgtctcc

SEQ ID NO: 27 - protein, 754 aa, Artificial Sequence
  HEA4(HSF-1) chimeric transcription factor
MVSKLSQLQTELLAALLESGLSKEALIQALGEPGPYLLAGEGPLDKGESCGGGRGELAELPNGLGETRGSEDETDDDGEDFTPPILKELENLSPEEAAHQKAVVETLLQEDPWRVAKMVKSYLQQHNIPQREVVDTTGLNQSHLSQHLNKGTPMKTQKRAALYTWYVRKQREVAQQFTHAGQGGLIEEPTGDELPTKKGRRNRFKWGPASQQILFQAYERQKNPSKEERETLVEECNRAECIQRGVSPSQAQGLGSNLVTEVRVYNWFANRRKEEAFRHKLSAGDMRAANLWPSPLMIKRSKKNSLALSLTADQMVSALLDAEPPILYSEYDPTRPFSEASMMGLLTNLADRELVHMINWAKRVPGFVDLTLHDQVHLLECAWLEILMIGLVWRSMEHPVKLLFAPNLLLDRNQGKCVEGMVEIFDMLLATSSRFRMMNLQGEEFVCLKSIILLNSGVYTFLSSTLKSLEEKDHIHRVLDKITDTLIHLMAKAGLTLQQQHQRLAQLLLILSHIRHMSNKGMEHLYSMKCKNVVPLYDLLLEAADAHRLHAPTSRGGASVEETDQSHLATAGSTSSHSLQKYYITGEAEGFPATVEKCLSVACLDKNELSDHLDAMDSNLDNLQTMLSSHGFSVDTSALLDLFSPSVTVPDMSLPDLDSSLASIQELLSPQEPPRPPEAENSSPDSGKQLVHYTAQPLFLLDPGSVDTGSNDLPVLFELGEGSYFSEGDGFAEDPTISLLTGSEPPKAKDPTVS

SEQ ID NO: 28 - DNA, 1887 bp, Unknown
  HEA4(Arnt) chimeric transcription factor
atggtgtccaagctgtcccagctgcagacagaactgctggcagcactgctggaaagcggcctgagcaaagaggccctgattcaggcactcggcgaacctggaccttatctgctcgctggcgaaggccctctggataagggcgagagctgtggcggaggaagaggagagctggccgagctgcctaacggcctgggcgagacaagaggcagcgaggacgagacagacgacgacggcgaggacttcaccccccccatcctgaaagagctggaaaacctgagccccgaggaagccgcccaccagaaagccgtggtggagacactgctgcaggaagatccctggcgggtcgccaagatggtcaagagctacctgcagcagcacaacatcccccagcgggaggtggtggacaccaccggcctgaaccagagccacctgagccagcacctgaacaagggcacccccatgaaaacccagaagagagccgccctgtacacttggtacgtgcggaagcagagagaggtggcccagcagtttacacacgccggccagggcggcctgatcgaggaacctaccggcgacgagctgcccaccaagaagggcagacggaaccggtttaagtggggccctgcatctcagcagatcctgttccaggcctacgagcggcagaagaaccccagcaaagaggaacgggagacactggtggaagagtgcaaccgggccgagtgcatccagagaggcgtgagcccttctcaggctcagggcctcggcagcaatctggtcaccgaagtgcgggtgtacaattggttcgccaaccggcggaaagaggaagccttccggcacaagctgtctgctggcgatatgagagccgccaacctgtggcccagccccctgatgatcaagcggagcaagaagaacagcctggccctgagcctgaccgccgatcagatggtgtccgctctgctggacgccgagccccctatcctgtacagcgagtacgaccccaccagacccttcagcgaggccagcatgatgggcctgctgaccaacctggccgaccgggagctggtgcacatgatcaactgggccaagcgggtgcccggcttcgtggacctgaccctgcacgaccaggtccacctgctggaatgtgcctggctggaaatcctgatgatcggcctcgtgtggagaagcatggaacaccccgtgaagctgctgttcgcccccaacctgctcctggaccggaaccagggaaagtgcgtggagggcatggtggagatcttcgacatgctgctggccacctccagccggttccggatgatgaacctgcagggcgaggaattcgtgtgcctgaagtccatcatcctgctgaacagcggcgtgtacaccttcctgtcatccaccctgaagtccctggaagagaaggaccacatccaccgggtgctggacaagatcaccgacaccctgatccacctgatggccaaggctggcctgacactccagcagcagcaccagagactggcccagctgctgctgatcctgagccacatccggcacatgagcaacaagggaatggaacacctgtacagcatgaagtgcaagaacgtggtgcccctgtacgacctgctgctcgaggctgccgatgcccacagactgcacgcccctacaagcagaggcggagccagcgtggaggaaaccgaccagtctcacctggccaccgccggcagcacaagcagccacagcctgcagaagtactacatcaccggcgaggccgagggattccctgccaccgtgcctgaggtcttccaggagatgctgtccatgctgggagatcagagcaacagctacaacaatgaagaattccctgatctaactatgtttccccccttttcagaa

SEQ ID NO: 29 - protein, 629 aa, Artificial Sequence
  HEA4(Arnt) chimeric transcription factor
MVSKLSQLQTELLAALLESGLSKEALIQALGEPGPYLLAGEGPLDKGESCGGGRGELAELPNGLGETRGSEDETDDDGEDFTPPILKELENLSPEEAAHQKAVVETLLQEDPWRVAKMVKSYLQQHNIPQREVVDTTGLNQSHLSQHLNKGTPMKTQKRAALYTWYVRKQREVAQQFTHAGQGGLIEEPTGDELPTKKGRRNRFKWGPASQQILFQAYERQKNPSKEERETLVEECNRAECIQRGVSPSQAQGLGSNLVTEVRVYNWFANRRKEEAFRHKLSAGDMRAANLWPSPLMIKRSKKNSLALSLTADQMVSALLDAEPPILYSEYDPTRPFSEASMMGLLTNLADRELVHMINWAKRVPGFVDLTLHDQVHLLECAWLEILMIGLVWRSMEHPVKLLFAPNLLLDRNQGKCVEGMVEIFDMLLATSSRFRMMNLQGEEFVCLKSIILLNSGVYTFLSSTLKSLEEKDHIHRVLDKITDTLIHLMAKAGLTLQQQHQRLAQLLLILSHIRHMSNKGMEHLYSMKCKNVVPLYDLLLEAADAHRLHAPTSRGGASVEETDQSHLATAGSTSSHSLQKYYITGEAEGFPATVPEVFQEMLSMLGDQSNSYNNEEFPDLTMFPPFSE

SEQ ID NO: 30 - DNA, 1074 bp, Unknown
  EGFRt nucleotide sequence
atgcttctcctggtgacaagccttctgctctgtgagttaccacacccagcattcctcctgatcccacgcaaagtgtgtaacggaataggtattggtgaatttaaagactcactctccataaatgctacgaatattaaacacttcaaaaactgcacctccatcagtggcgatctccacatcctgccggtggcatttaggggtgactccttcacacatactcctcctctggatccacaggaactggatattctgaaaaccgtaaaggaaatcacagggtttttgctgattcaggcttggcctgaaaacaggacggacctccatgcctttgagaacctagaaatcatacgcggcaggaccaagcaacatggtcagttttctcttgcagtcgtcagcctgaacataacatccttgggattacgctccctcaaggagataagtgatggagatgtgataatttcaggaaacaaaaatttgtgctatgcaaatacaataaactggaaaaaactgtttgggacctccggtcagaaaaccaaaattataagcaacagaggtgaaaacagctgcaaggccacaggccaggtctgccatgccttgtgctcccccgagggctgctggggcccggagcccagggactgcgtctcttgccggaatgtcagccgaggcagggaatgcgtggacaagtgcaaccttctggagggtgagccaagggagtttgtggagaactctgagtgcatacagtgccacccagagtgcctgcctcaggccatgaacatcacctgcacaggacggggaccagacaactgtatccagtgtgcccactacattgacggcccccactgcgtcaagacctgcccggcaggagtcatgggagaaaacaacaccctggtctggaagtacgcagacgccggccatgtgtgccacctgtgccatccaaactgcacctacggatgcactgggccaggtcttgaaggctgtccaacgaatgggcctaagatcccgtccatcgccactgggatggtgggggccctcctcttgctgctggtggtggccctggggatcggcctcttcatgtga

SEQ ID NO: 31 - protein, 357 aa, Artificial Sequence
  EGFRt amino acid sequence
  EGFRt amino acid sequence
MLLLVTSLLLCELPHPAFLLIPRKVCNGIGIGEFKDSLSINATNIKHFKNCTSISGDLHILPVAFRGDSFTHTPPLDPQELDILKTVKEITGFLLIQAWPENRTDLHAFENLEIIRGRTKQHGQFSLAVVSLNITSLGLRSLKEISDGDVIISGNKNLCYANTINWKKLFGTSGQKTKIISNRGENSCKATGQVCHALCSPEGCWGPEPRDCVSCRNVSRGRECVDKCNLLEGEPREFVENSECIQCHPECLPQAMNITCTGRGPDNCIQCAHYIDGPHCVKTCPAGVMGENNTLVWKYADAGHVCHLCHPNCTYGCTGPGLEGCPTNGPKIPSIATGMVGALLLLLVVALGIGLFM

SEQ ID NO: 32 - DNA, 408 bp, Unknown
  Her2t
atgcttctcctggtgacaagccttctgctctgtgagttaccacacccagcattcctcctgatcccatgccaccctgagtgtcagccccagaatggctcagtgacctgttttggaccggaggctgaccagtgtgtggcctgtgcccactataaggaccctcccttctgcgtggcccgctgccccagcggtgtgaaacctgacctctcctacatgcccatctggaagtttccagatgaggagggcgcatgccagccttgccccatcaactgcacccactcctgtgtggacctggatgacaagggctgccccgccgagcagagagccagccctctgacgtccatcatctctgcggtggttggcattctgctggtcgtggtcttgggggtggtctttgggatcctcatctga

SEQ ID NO: 33 - protein, 135 aa, Artificial Sequence
  Her2t
MLLLVTSLLLCELPHPAFLLIPCHPECQPQNGSVTCFGPEADQCVACAHYKDPPFCVARCPSGVKPDLSYMPIWKFPDEEGACQPCPINCTHSCVDLDDKGCPAEQRASPLTSIISAVVGILLVVVLGVVFGILI

SEQ ID NO: 34 - DNA, 429 bp, Unknown
  Her2tG
atgcttctcctggtgacaagccttctgctctgtgagttaccacacccagcattcctcctgatcccatgccaccctgagtgtcagccccagaatggctcagtgacctgttttggaccggaggctgaccagtgtgtggcctgtgcccactataaggaccctcccttctgcgtggcccgctgccccagcggtgtgaaacctgacctctcctacatgcccatctggaagtttccagatgaggagggcgcatgccagccttgccccatcaactgcacccactcctgtgtggacctggatgacaagggctgccccgccgagcagagagccagcccgttaacgggtggaggcagcggaggtggctccatcatctctgcggtggttggcattctgctggtcgtggtcttgggggtggtctttgggatcctcatctga

SEQ ID NO: 35 - protein, 142 aa, Artificial Sequence
  Her2tG
MLLLVTSLLLCELPHPAFLLIPCHPECQPQNGSVTCFGPEADQCVACAHYKDPPFCVARCPSGVKPDLSYMPIWKFPDEEGACQPCPINCTHSCVDLDDKGCPAEQRASPLTGGGSGGGSIISAVVGILLVVVLGVVFGILI

SEQ ID NO: 36 - DNA, 972 bp, Unknown
  CD19t
atgccacctcctcgcctcctcttcttcctcctcttcctcacccccatggaagtcaggcccgaggaacctctagtggtgaaggtggaagagggagataacgctgtgctgcagtgcctcaaggggacctcagatggccccactcagcagctgacctggtctcgggagtccccgcttaaacccttcttaaaactcagcctggggctgccaggcctgggaatccacatgaggcccctggccatctggcttttcatcttcaacgtctctcaacagatggggggcttctacctgtgccagccggggcccccctctgagaaggcctggcagcctggctggacagtcaatgtggagggcagcggggagctgttccggtggaatgtttcggacctaggtggcctgggctgtggcctgaagaacaggtcctcagagggccccagctccccttccgggaagctcatgagccccaagctgtatgtgtgggccaaagaccgccctgagatctgggagggagagcctccgtgtgtcccaccgagggacagcctgaaccagagcctcagccaggacctcaccatggcccctggctccacactctggctgtcctgtggggtaccccctgactctgtgtccaggggccccctctcctggacccatgtgcaccccaaggggcctaagtcattgctgagcctagagctgaaggacgatcgcccggccagagatatgtgggtaatggagacgggtctgttgttgccccgggccacagctcaagacgctggaaagtattattgtcaccgtggcaacctgaccatgtcattccacctggagatcactgctcggccagtactatggcactggctgctgaggactggtggctggaaggtctcagctgtgactttggcttatctgatcttctgcctgtgttcccttgtgggcattcttcatcttcaaagagccctggtcctgaggaggaaaagataa

SEQ ID NO: 37 - protein, 323 aa, Artificial Sequence
  CD19t
MPPPRLLFFLLFLTPMEVRPEEPLVVKVEEGDNAVLQCLKGTSDGPTQQLTWSRESPLKPFLKLSLGLPGLGIHMRPLAIWLFIFNVSQQMGGFYLCQPGPPSEKAWQPGWTVNVEGSGELFRWNVSDLGGLGCGLKNRSSEGPSSPSGKLMSPKLYVWAKDRPEIWEGEPPCVPPRDSLNQSLSQDLTMAPGSTLWLSCGVPPDSVSRGPLSWTHVHPKGPKSLLSLELKDDRPARDMWVMETGLLLPRATAQDAGKYYCHRGNLTMSFHLEITARPVLWHWLLRTGGWKVSAVTLAYLIFCLCSLVGILHLQRALVLRRKR

SEQ ID NO: 38 - DNA, 561 bp, Unknown
  DHFRdm
atggttggttcgctaaactgcatcgtcgctgtgtcccagaacatgggcatcggcaagaacggggacttcccctggccaccgctcaggaatgaatccagatatttccagagaatgaccacaacctcttcagtagaaggtaaacagaatctggtgattatgggtaagaagacctggttctccattcctgagaagaatcgacctttaaagggtagaattaatttagttctcagcagagaactcaaggaacctccacaaggagctcattttctttccagaagtctagatgatgccttaaaacttactgaacaaccagaattagcaaataaagtagacatggtctggatagttggtggcagttctgtttataaggaagccatgaatcacccaggccatcttaaactatttgtgacaaggatcatgcaagactttgaaagtgacacgttttttccagaaattgatttggagaaatataaacttctgccagaatacccaggtgttctctctgatgtccaggaggagaaaggcattaagtacaaatttgaagtatatgagaagaatgat

SEQ ID NO: 39 - protein, 186 aa, Artificial Sequence
  DHFRdm
VGSLNCIVAVSQNMGIGKNGDFPWPPLRNESRYFQRMTTTSSVEGKQNLVIMGKKTWFSIPEKNRPLKGRINLVLSRELKEPPQGAHFLSRSLDDALKLTEQPELANKVDMVWIVGGSSVYKEAMNHPGHLKLFVTRIMQDFESDTFFPEIDLEKYKLLPEYPGVLSDVQEEKGIKYKFEVYEKND

SEQ ID NO: 40 - DNA, 804 bp, Unknown
  huCD19 scFv (G01S)
atgcttctcctggtgacaagccttctgctctgtgagttaccacacccagcattcctcctgatcccagaggtgcagctggtcgaatccggaggaggactggtccagcccggccggagcctgagactgagctgtgccgcttccggattcacttttgacgattacgcaatgcattgggtgaggcaggcccctggcaaggggctggaatgggtctccggaatctcttggaacagtgggcgcattggatatgccgattctgtgaagggccgattcactatctctcgggacaacgctaaaaatagtctgtttctgcagatgaattccctgcgcgccgaggataccgccgtgtactattgcgcccgagaccagggctaccactactatgatagcgccgaacatgcattcgacatttggggacagggaactgtggtcaccgtgagctccggaggaggaggaagcggaggaggagggtccggaggcgggggatcacagagcgcactgacccagccacggagcgtgagcggatttcctgggcagtctgtcaccattagttgcacaggcaccacatcagacgatgtgagctggtaccagcagcacccagggaaggctccccagctgatgctgtatgacgtgtccaaaagaccttctggcgtcccacataggtttagtggaagccggagcggccgggcagccagtctgatcatttcagggctgcagacagaggacgaagctgattatttctgttctagttacgcaggcagatataactctgtgctgtttggcgggggaacaaagctgactgtcctg

SEQ ID NO: 41 - protein, 268 aa, Artificial Sequence
  huCD19 scFv (G01S)
MLLLVTSLLLCELPHPAFLLIPEVQLVESGGGLVQPGRSLRLSCAASGFTFDDYAMHWVRQAPGKGLEWVSGISWNSGRIGYADSVKGRFTISRDNAKNSLFLQMNSLRAEDTAVYYCARDQGYHYYDSAEHAFDIWGQGTVVTVSSGGGGSGGGGSGGGGSQSALTQPRSVSGFPGQSVTISCTGTTSDDVSWYQQHPGKAPQLMLYDVSKRPSGVPHRFSGSRSGRAASLIISGLQTEDEADYFCSSYAGRYNSVLFGGGTKLTVL

SEQ ID NO: 42 - DNA, 801 bp, Unknown
  muCD19 (FMC63) scFv
atgctgctgctggtgaccagcctgctgctgtgcgagctgccccaccccgcctttctgctgatccccgacatccagatgacccagaccacctccagcctgagcgccagcctgggcgaccgggtgaccatcagctgccgggccagccaggacatcagcaagtacctgaactggtatcagcagaagcccgacggcaccgtcaagctgctgatctaccacaccagccggctgcacagcggcgtgcccagccggtttagcggcagcggctccggcaccgactacagcctgaccatctccaacctggaacaggaagatatcgccacctacttttgccagcagggcaacacactgccctacacctttggcggcggaacaaagctggaaatcaccggcagcacctccggcagcggcaagcctggcagcggcgagggcagcaccaagggcgaggtgaagctgcaggaaagcggccctggcctggtggcccccagccagagcctgagcgtgacctgcaccgtgagcggcgtgagcctgcccgactacggcgtgagctggatccggcagccccccaggaagggcctggaatggctgggcgtgatctggggcagcgagaccacctactacaacagcgccctgaagagccggctgaccatcatcaaggacaacagcaagagccaggtgttcctgaagatgaacagcctgcagaccgacgacaccgccatctactactgcgccaagcactactactacggcggcagctacgccatggactactggggccagggcaccagcgtgaccgtgagcagc

SEQ ID NO: 43 - protein, 267 aa, Artificial Sequence
  muCD19 (FMC63) scFv
MLLLVTSLLLCELPHPAFLLIPDIQMTQTTSSLSASLGDRVTISCRASQDISKYLNWYQQKPDGTVKLLIYHTSRLHSGVPSRFSGSGSGTDYSLTISNLEQEDIATYFCQQGNTLPYTFGGGTKLEITGSTSGSGKPGSGEGSTKGEVKLQESGPGLVAPSQSLSVTCTVSGVSLPDYGVSWIRQPPRKGLEWLGVIWGSETTYYNSALKSRLTIIKDNSKSQVFLKMNSLQTDDTAIYYCAKHYYYGGSYAMDYWGQGTSVTVSS

SEQ ID NO: 44 - DNA, 798 bp, Unknown
  CD20 (Leu16) scFv
atggagacagacacactcctgctatgggtgctgctgctctgggttccaggttccacaggtgacattgtgctgacccaatctccagctatcctgtctgcatctccaggggagaaggtcacaatgacttgcagggccagctcaagtgtaaattacatggactggtaccagaagaagccaggatcctcccccaaaccctggatttatgccacatccaacctggcttctggagtccctgctcgcttcagtggcagtgggtctgggacctcttactctctcacaatcagcagagtggaggctgaagatgctgccacttattactgccagcagtggagttttaatccacccacgttcggaggggggaccaagctggaaataaaaggcagtactagcggtggtggctccgggggcggttccggtgggggcggcagcagcgaggtgcagctgcagcagtctggggctgagctggtgaagcctggggcctcagtgaagatgtcctgcaaggcttctggctacacatttaccagttacaatatgcactgggtaaagcagacacctggacagggcctggaatggattggagctatttatccaggaaatggtgatacttcctacaatcagaagttcaaaggcaaggccacattgactgcagacaaatcctccagcacagcctacatgcagctcagcagcctgacatctgaggactctgcggactattactgtgcaagatctaattattacggtagtagctactggttcttcgatgtctggggcgcagggaccacggtcaccgtctcctca

SEQ ID NO: 45 - protein, 266 aa, Artificial Sequence
  CD20 (Leu16) scFv
METDTLLLWVLLLWVPGSTGDIVLTQSPAILSASPGEKVTMTCRASSSVNYMDWYQKKPGSSPKPWIYATSNLASGVPARFSGSGSGTSYSLTISRVEAEDAATYYCQQWSFNPPTFGGGTKLEIKGSTSGGGSGGGSGGGGSSEVQLQQSGAELVKPGASVKMSCKASGYTFTSYNMHWVKQTPGQGLEWIGAIYPGNGDTSYNQKFKGKATLTADKSSSTAYMQLSSLTSEDSADYYCARSNYYGSSYWFFDVWGAGTTVTVSS

SEQ ID NO: 46 - DNA, 810 bp, Unknown
  CD22 (m971) scFv
atgcttctcctggtgacaagccttctgctctgtgagttaccacacccagcattcctcctgatcccacaggtacagctgcagcagtcaggtccaggactggtgaagccctcgcagaccctctcactcacctgtgccatctccggggacagtgtctctagcaacagtgctgcttggaactggatcaggcagtccccatcgagaggccttgagtggctgggaaggacatactacaggtccaagtggtataatgattatgcagtatctgtgaaaagtcgaataaccatcaacccagacacatccaagaaccagttctccctgcagctgaactctgtgactcccgaggacacggctgtgtattactgtgcaagagaagtgactggggatctcgaggatgcttttgatatctggggccaagggacaatggtcaccgtctcctcaggcggagggggctctggcggcggaggatctgggggagggggcagcgacatccagatgacccagtctccatcgtccctgtctgcatctgtaggagacagagtcaccatcacttgccgggcaagccagaccatttggagctacttaaattggtatcagcagagaccagggaaagcccctaacctcctgatctatgctgcatccagtttgcaaagtggggtcccatcaaggttcagtggcaggggatctgggacagatttcactctcaccatcagcagtctgcaagctgaagattttgcaacttactactgtcaacagagttacagtatccctcagacttttggccaggggaccaagctggagatcaaacgaact

SEQ ID NO: 47 - protein, 270 aa, Artificial Sequence
  CD22 (m971) scFv
MLLLVTSLLLCELPHPAFLLIPQVQLQQSGPGLVKPSQTLSLTCAISGDSVSSNSAAWNWIRQSPSRGLEWLGRTYYRSKWYNDYAVSVKSRITINPDTSKNQFSLQLNSVTPEDTAVYYCAREVTGDLEDAFDIWGQGTMVTVSSGGGGSGGGGSGGGGSDIQMTQSPSSLSASVGDRVTITCRASQTIWSYLNWYQQRPGKAPNLLIYAASSLQSGVPSRFSGRGSGTDFTLTISSLQAEDFATYYCQQSYSIPQTFGQGTKLEIKRT

SEQ ID NO: 48 - DNA, 948 bp, Unknown
  B7H3 (hBRCA84D) scFv
atgctgcgtcggcggggcagccctggcatgggtgtgcatgtgggtgcagccctgggagcactgtggttctgcctcacaggagccctggaggtccaggtccctgaagacccagtggtggcactggtgggcaccgatgccaccctgtgctgctccttctcccctgagcctggcttcagcctggcacagctcaacctcatctggcagctgacagataccaaacagctggtgcacagctttgctgagggccaggaccagggcagcgcctatgccaaccgcacggccctcttcccggacctgctggcacagggcaacgcatccctgaggctgcagcgcgtgcgtgtggcggacgagggcagcttcacctgcttcgtgagcatccgggatttcggcagcgctgccgtcagcctgcaggtggccgctccctactcgaagcccagcatgaccctggagcccaacaaggacctgcggccaggggacacggtgaccatcacgtgctccagctaccagggctaccctgaggctgaggtgttctggcaggatgggcagggtgtgcccctgactggcaacgtgaccacgtcgcagatggccaacgagcagggcttgtttgatgtgcacagcatcctgcgggtggtgctgggtgcaaatggcacctacagctgcctggtgcgcaaccccgtgctgcagcaggatgcgcacagctctgtcaccatcacagggcagcctatgacattccccccagaggccctgtgggtgaccgtggggctgtctgtctgtctcattgcactgctggtggccctggctttcgtgtgctggagaaagatcaaacagagctgtgaggaggagaatgcaggagctgaggaccaggatggggagggagaaggctccaagacagccctgcagcctctgaaacactctgacagcaaagaagatgatggacaagaaatagcc

SEQ ID NO: 49 - protein, 316 aa, Artificial Sequence
  B7H3 (hBRCA84D) scFv
MLRRRGSPGMGVHVGAALGALWFCLTGALEVQVPEDPVVALVGTDATLCCSFSPEPGFSLAQLNLIWQLTDTKQLVHSFAEGQDQGSAYANRTALFPDLLAQGNASLRLQRVRVADEGSFTCFVSIRDFGSAAVSLQVAAPYSKPSMTLEPNKDLRPGDTVTITCSSYQGYPEAEVFWQDGQGVPLTGNVTTSQMANEQGLFDVHSILRVVLGANGTYSCLVRNPVLQQDAHSSVTITGQPMTFPPEALWVTVGLSVCLIALLVALAFVCWRKIKQSCEEENAGAEDQDGEGEGSKTALQPLKHSDSKEDDGQEIA

SEQ ID NO: 50 - DNA, 792 bp, Unknown
  L1CAM (CE7) scFv
atgctgctgctggtgaccagcctgctgctgtgcgagctgccccaccccgcctttctgctgatcccccaggtgcagctgcagcagcctggcgccgagctggtgaagccaggcgccagcgtgaagctgtcctgcaaggccagcggctacaccttcaccggctactggatgcactgggtgaagcagagacccggccacggcctggaatggatcggcgagatcaaccccagcaacggccggaccaactacaacgagcggttcaagagcaaggccaccctgaccgtggacaagagcagcaccaccgccttcatgcagctgtccggcctgaccagcgaggacagcgccgtgtacttctgcgccagggactactacggcaccagctacaacttcgactactggggccagggcaccacactgaccgtgagcagcggcggagggggctctggcggcggaggatctgggggagggggcagcgacatccagatgacccagagcagcagcagcttcagcgtgagcctgggcgaccgggtgaccatcacctgtaaggccaacgaggacatcaacaaccggctggcctggtatcagcagacccccggcaacagccccaggctgctgatcagcggcgccaccaacctggtgaccggcgtgcccagccggtttagcggcagcggctccggcaaggactacaccctgaccatcacaagcctgcaggccgaggacttcgccacctactactgccagcagtactggtccacccccttcaccttcggcagcggcaccgagctggaaatcaaa

SEQ ID NO: 51 - protein, 264 aa, Artificial Sequence
  L1CAM (CE7) scFv
MLLLVTSLLLCELPHPAFLLIPQVQLQQPGAELVKPGASVKLSCKASGYTFTGYWMHWVKQRPGHGLEWIGEINPSNGRTNYNERFKSKATLTVDKSSTTAFMQLSGLTSEDSAVYFCARDYYGTSYNFDYWGQGTTLTVSSGGGGSGGGGSGGGGSDIQMTQSSSSFSVSLGDRVTITCKANEDINNRLAWYQQTPGNSPRLLISGATNLVTGVPSRFSGSGSGKDYTLTITSLQAEDFATYYCQQYWSTPFTFGSGTELEIK

SEQ ID NO: 52 - DNA, 795 bp, Unknown
  EGFR (cetuximab) scFv
atgcttctcctggtgacaagccttctgctctgtgagttaccacacccagcattcctcctgatcccacaggtgcagctgaaacagagcggcccgggcctggtgcagccgagccagagcctgagcattacctgcaccgtgagcggctttagcctgaccaactatggcgtgcattgggtgcgccagagcccgggcaaaggcctggaatggctgggcgtgatttggagcggcggcaacaccgattataacaccccgtttaccagccgcctgagcattaacaaagataacagcaaaagccaggtgttttttaaaatgaacagcctgcagagcaacgataccgcgatttattattgcgcgcgcgcgctgacctattatgattatgaatttgcgtattggggccagggcaccctggtgaccgtgagcgcgggcggcggcggcagcggcggcggcggcagcggcggcggcggcagcgatattctgctgacccagagcccggtgattctgagcgtgagcccgggcgaacgcgtgagctttagctgccgcgcgagccagagcattggcaccaacattcattggtatcagcagcgcaccaacggcagcccgcgcctgctgattaaatatgcgagcgaaagcattagcggcattccgagccgctttagcggcagcggcagcggcaccgattttaccctgagcattaacagcgtggaaagcgaagatattgcggattattattgccagcagaacaacaactggccgaccacctttggcgcgggcaccaaactggaactgaaacgcacc

SEQ ID NO: 53 - protein, 265 aa, Artificial Sequence
  EGFR scFv
MLLLVTSLLLCELPHPAFLLIPQVQLKQSGPGLVQPSQSLSITCTVSGFSLTNYGVHWVRQSPGKGLEWLGVIWSGGNTDYNTPFTSRLSINKDNSKSQVFFKMNSLQSNDTAIYYCARALTYYDYEFAYWGQGTLVTVSAGGGGSGGGGSGGGGSDILLTQSPVILSVSPGERVSFSCRASQSIGTNIHWYQQRTNGSPRLLIKYASESISGIPSRFSGSGSGTDFTLSINSVESEDIADYYCQQNNNWPTTFGAGTKLELKRT

SEQ ID NO: 54 - DNA, 792 bp, Unknown
  EGFRVIII (806) scFv
atgctgctgctggtgacaagcctgctgctgtgcgagctgccacaccctgctttcctgctgatccctgatgtgcagctgcaggaatcaggcccaagcctggtcaaaccctcccagtctctgagtctgacctgtacagtgactgggtactccatcacatctgatttcgcatggaactggattaggcagtttccaggcaataagctggagtggatgggctacatctcatatagcgggaacactcgctataatcccagtctgaaatcacggatcagcattactagagacaccagcaagaaccagttctttctgcagctgaattccgtgaccattgaggataccgccacatactattgcgtcacagctggcagaggctttccatactggggacagggcacactggtgactgtcagcgccggctccacctctgggagtggaaaacctggctccggggaaggatctacaaagggagacatcctgatgactcagtccccaagctccatgtcagtgagcctgggcgacaccgtctctattacatgtcactctagtcaggatatcaacagtaatattggctggctgcagcagcgacccggcaagtctttcaaagggctgatctatcatggaactaacctggacgatgaagtgcctagcagattttccggctctgggagtggagctgattacagtctgaccatttcaagcctggagtcagaagacttcgcagattactattgcgtccagtatgcccagttcccctggacttttggcgggggaaccaagctggagatcaaacgg

SEQ ID NO: 55 - protein, 264 aa, Artificial Sequence
  EGFRVIII (806) scFv
MLLLVTSLLLCELPHPAFLLIPDVQLQESGPSLVKPSQSLSLTCTVTGYSITSDFAWNWIRQFPGNKLEWMGYISYSGNTRYNPSLKSRISITRDTSKNQFFLQLNSVTIEDTATYYCVTAGRGFPYWGQGTLVTVSAGSTSGSGKPGSGEGSTKGDILMTQSPSSMSVSLGDTVSITCHSSQDINSNIGWLQQRPGKSFKGLIYHGTNLDDEVPSRFSGSGSGADYSLTISSLESEDFADYYCVQYAQFPWTFGGGTKLEIKR

SEQ ID NO: 56 - DNA, 777 bp, Unknown
  EphA2 (2A4) scFv
atgcttctcctggtgacaagccttctgctctgtgagttaccacacccagcattcctcctgatcccacaggtgcagctgttggagtctgggggaggcttggtacagcctggggggtccctgagactctcctgtgcagcctctggattcacctttagcagctataccatgtcttgggtgcgacaggcccctggacaagcgcttgagtggatgggaaccattagtagtcgtggtacttacacctactatccagacagtgtgaagggccgattcaccatctccagagacaacgccaagaactcactgtatctgcaaatgaacagcctgagagccgaggacacggctgtgtattactgtgcgagagaagctatctttactcactggggccgtggcaccctggtcaccgtctcctcaggtggtggtggttctggcggcggcggctccggtggtggtggttctgacatccagttgacccagtctccatcctccctgtctgcatctgtaggagacagagtcaccatcacttgcaaggcgagtcaggacattaataactatcacagctggtaccagcagaaacctggccaggctcccaggctcctcatctatcgtgcaaacagattggtcgatggggtcccagacaggttcagtggcagcgggtatggaacagattttaccctcacaattaataacatagaatctgaggatgctgcatattacttctgtctgaaatataatgtgtttccgtacacgttcggccaagggaccaaggtggagatcaaa

SEQ ID NO: 57 - protein, 259 aa, Artificial Sequence
  EphA2 (2A4) scFv
MLLLVTSLLLCELPHPAFLLIPQVQLLESGGGLVQPGGSLRLSCAASGFTFSSYTMSWVRQAPGQALEWMGTISSRGTYTYYPDSVKGRFTISRDNAKNSLYLQMNSLRAEDTAVYYCAREAIFTHWGRGTLVTVSSGGGGSGGGGSGGGGSDIQLTQSPSSLSASVGDRVTITCKASQDINNYHSWYQQKPGQAPRLLIYRANRLVDGVPDRFSGSGYGTDFTLTINNIESEDAAYYFCLKYNVFPYTFGQGTKVEIK

SEQ ID NO: 58 - DNA, 777 bp, Unknown
  EpHA2 (4H5) scFv
atgcttctcctggtgacaagccttctgctctgtgagttaccacacccagcattcctcctgatcccacaggtgcagctgttggagtctgggggaggcttggtacagcctggggggtccctgagactctcctgtgcagcctctggattcacctttagcagctataccatgtcttgggtgcgacaggcccctggacaagcgcttgagtggatgggaaccattagtagtggtggtacttacacctactatccagacagtgtgaagggccgattcaccatctccagagacaacgccaagaactcactgtatctgcaaatgaacagcctgagagccgaggacacggctgtgtattactgtgcgagagaagctatctttacttactggggccgtggcaccctggtcaccgtctcctcaggtggtggtggttctggcggcggcggctccggtggtggtggttctgacatccagttgacccagtctccatcctccctgtctgcatctgtaggagacagagtcaccatcacttgcaaggcgagtcaggacattaataactatttaagctggtaccagcagaaacctggccaggctcccaggctcctcatctatcgtgcaaacagattggtagatggggtcccagacaggttcagtggcagcgggtatggaacagattttaccctcacaattaataacatagaatctgaggatgctgcatattacttctgtctgaaatatgatgtgtttccgtacacgttcggccaagggaccaaggtggagatcaaa

SEQ ID NO: 59 - protein, 259 aa, Artificial Sequence
  EpHA2 (4H5) scFv
MLLLVTSLLLCELPHPAFLLIPQVQLLESGGGLVQPGGSLRLSCAASGFTFSSYTMSWVRQAPGQALEWMGTISSGGTYTYYPDSVKGRFTISRDNAKNSLYLQMNSLRAEDTAVYYCAREAIFTYWGRGTLVTVSSGGGGSGGGGSGGGGSDIQLTQSPSSLSASVGDRVTITCKASQDINNYLSWYQQKPGQAPRLLIYRANRLVDGVPDRFSGSGYGTDFTLTINNIESEDAAYYFCLKYDVFPYTFGQGTKVEIK

SEQ ID NO: 60 - DNA, 819 bp, Unknown
  FITC (E2) scFv
atgcttctcctggtgacaagccttctgctctgtgagttaccacacccagcattcctcctgatcccaagcgtgctgacacagcctagctccgtgtctgccgcccctggccagaaagtgaccatcagctgtagcggcagcaccagcaacatcggcaacaactacgtgtcctggtatcagcagcaccccggcaaggcccccaagctgatgatctacgacgtgtccaagcggcccagcggcgtgcccgatagattttccggcagcaagagcggcaacagcgccagcctggatatcagcggcctgcagtctgaggacgaggccgactactattgcgccgcctgggacgatagcctgagcgagttcctgtttggcaccggcaccaagctgacagtgctgggcggaggcggaggatctggcggcggaggaagtggcggagggggatctcaggtgcagctggtggaaagcggcggcaacctggtgcagcctggcggatctctgagactgagctgtgccgccagcggcttcaccttcggcagcttcagcatgagctgggtgcgccaggctcctgggggaggactggaatgggtggcaggactgagcgccagaagcagcctgacccactacgccgatagcgtgaagggccggttcaccatcagccgggacaacgccaagaacagcgtgtacctgcagatgaacagcctgcgggtggaagataccgccgtgtactactgcgccagacggtcctacgacagcagcggctactggggccacttctacagctacatggacgtgtggggccagggcaccctcgtgacagtgtct

SEQ ID NO: 61 - protein, 273 aa, Artificial Sequence
  FITC (E2) scFv
MLLLVTSLLLCELPHPAFLLIPSVLTQPSSVSAAPGQKVTISCSGSTSNIGNNYVSWYQQHPGKAPKLMIYDVSKRPSGVPDRFSGSKSGNSASLDISGLQSEDEADYYCAAWDDSLSEFLFGTGTKLTVLGGGGGSGGGGSGGGGSQVQLVESGGNLVQPGGSLRLSCAASGFTFGSFSMSWVRQAPGGGLEWVAGLSARSSLTHYADSVKGRFTISRDNAKNSVYLQMNSLRVEDTAVYYCARRSYDSSGYWGHFYSYMDVWGQGTLVTVS

SEQ ID NO: 62 - DNA, 381 bp, Unknown
  GD2 (hu3F8) scFv
atgcttctcctggtgacaagccttctgctctgtgagttaccacacccagcattcctcctgatcccaagcatcgtgatgacccagacccccaagttcctgctggtgagcgccggcgacagggtgaccatcacctgcaaggccagccagagcgtgagcaacgacgtgacctggtaccagcagaaggccggccagagccccaagctgctgatctacagcgccagcaacaggtacagcggcgtgcccgacaggttcaccggcagcggctacggcaccgccttcaccttcaccatcagcaccgtgcaggccgaggacctggccgtgtacttctgccagcaggactacagcagcttcggcggcggcaccaagctggagatcaagagg

SEQ ID NO: 63 - protein, 127 aa, Artificial Sequence
  GD2 (hu3F8) scFv
MLLLVTSLLLCELPHPAFLLIPSIVMTQTPKFLLVSAGDRVTITCKASQSVSNDVTWYQQKAGQSPKLLIYSASNRYSGVPDRFTGSGYGTAFTFTISTVQAEDLAVYFCQQDYSSFGGGTKLEIKR

SEQ ID NO: 64 - DNA, 801 bp, Unknown
  Her2 (Herceptin) scFv
atgcttctcctggtgacaagccttctgctctgtgagttaccacacccagcattcctcctgatcccagatatccagatgacccagtccccgagctccctgtccgcctctgtgggcgatagggtcaccatcacctgccgtgccagtcaggatgtgaatactgctgtagcctggtatcaacagaaaccaggaaaagctccgaaactactgatttactcggcatccttcctctactctggagtcccttctcgcttctctggttccagatctgggacggatttcactctgaccatcagcagtctgcagccggaagacttcgcaacttattactgtcagcaacattatactactcctcccacgttcggacagggtaccaaggtggagatcaaaggcagtactagcggcggtggctccgggggcggatccggtgggggcggcagcagcgaggttcagctggtggagtctggcggtggcctggtgcagccagggggctcactccgtttgtcctgtgcagcttctggcttcaacattaaagacacctatatacactgggtgcgtcaggccccgggtaagggcctggaatgggttgcaaggatttatcctacgaatggttatactagatatgccgatagcgtcaagggccgtttcactataagcgcagacacatccaaaaacacagcctacctgcagatgaacagcctgcgtgctgaggacactgccgtctattattgttctagatggggaggggacggcttctatgctatggactactggggtcaaggaaccctggtcaccgtctcgagt

SEQ ID NO: 65 - protein, 267 aa, Artificial Sequence
  Her2 (Herceptin) scFv
MLLLVTSLLLCELPHPAFLLIPDIQMTQSPSSLSASVGDRVTITCRASQDVNTAVAWYQQKPGKAPKLLIYSASFLYSGVPSRFSGSRSGTDFTLTISSLQPEDFATYYCQQHYTTPPTFGQGTKVEIKGSTSGGGSGGGSGGGGSSEVQLVESGGGLVQPGGSLRLSCAASGFNIKDTYIHWVRQAPGKGLEWVARIYPTNGYTRYADSVKGRFTISADTSKNTAYLQMNSLRAEDTAVYYCSRWGGDGFYAMDYWGQGTLVTVSS

SEQ ID NO: 66 - DNA, 722 bp, Unknown
  IL13R2a (hu08) VlVh scFv
atgcttctcctggtgacaagccttctgctctgtgagttaccacacccagcattcctcctgatcccagacatccagatgacccagtccccctcttctctgtctgcctctgtgggcgacagagtgaccatcacctgtaaggccagtcaggatgtaggtactgctgtagcctggtatcagcagaagcctggcaaggctcccaagctgctgatctactcggcatcctaccggtccactggcgtgccttccagattctccggctctggctctggcaccgatttcaccctgaccatctcctccctccagcctgaggatttcgccacctactactgccagcaccattatagtgctccgtggacgtttggcggcggaacaaaggtggagatcaagggtggtggtggttctggcggcggcggctccggtggtggtggttctgaggtgcagctggtggagtctggcggcggactggtgcagcctggcggctctctgagactgtcttgtgccgcctccggcttcaccttcagtaggaatggcatgtcttgggtgaggcaggcccctggcaagggcctggagtgggtggccaccgttagtagtggtggtagttacatctactatgcagacagtgtgaaggggcggttcaccatctccagggacaacgccaagaactccctgtacctccagatgaactccctgagggccgaggataccgccgtgtactactgtgc

SEQ ID NO: 67 - protein, 240 aa, Artificial Sequence
  IL13RA2 (HU08) VlVh scFv
MLLLVTSLLLCELPHPAFLLIPDIQMTQSPSSLSASVGDRVTITCKASQDVGTAVAWYQQKPGKAPKLLIYSASYRSTGVPSRFSGSGSGTDFTLTISSLQPEDFATYYCQHHYSAPWTFGGGTKVEIKGGGGSGGGGSGGGGSEVQLVESGGGLVQPGGSLRLSCAASGFTFSRNGMSWVRQAPGKGLEWVATVSSGGSYIYYADSVKGRFTISRDNAKNSLYLQMNSLRAEDTAVYYC

SEQ ID NO: 68 - DNA, 809 bp, Unknown
  IL13RA2 (HU08) VlVh scFv
atgcttctcctggtgacaagccttctgctctgtgagttaccacacccagcattcctcctgatcccagaggtgcagctggtggagtctggcggcggactggtgcagcctggcggctctctgagactgtcttgtgccgcctccggcttcaccttcagtaggaatggcatgtcttgggtgaggcaggcccctggcaagggcctggagtgggtggccaccgttagtagtggtggtagttacatctactatgcagacagtgtgaaggggcggttcaccatctccagggacaacgccaagaactccctgtacctccagatgaactccctgagggccgaggataccgccgtgtactactgtgccagacaagggactacggcactagctacgaggttcttcgatgtctggggccagggcaccctggtgaccgtgtcctctggtggtggtggttctggcggcggcggctccggtggtggtggttctgacatccagatgacccagtccccctcttctctgtctgcctctgtgggcgacagagtgaccatcacctgtaaggccagtcaggatgtaggtactgctgtagcctggtatcagcagaagcctggcaaggctcccaagctgctgatctactcggcatcctaccggtccactggcgtgccttccagattctccggctctggctctggcaccgatttcaccctgaccatctcctccctccagcctgaggatttcgccacctactactgccagcaccattatagtgctccgtggacgtttggcggcggaacaaaggtggagatcaaggaatctaagta

SEQ ID NO: 69 - protein, 269 aa, Artificial Sequence
  IL13RA2 (HU08) VlVh scFv
MLLLVTSLLLCELPHPAFLLIPEVQLVESGGGLVQPGGSLRLSCAASGFTFSRNGMSWVRQAPGKGLEWVATVSSGGSYIYYADSVKGRFTISRDNAKNSLYLQMNSLRAEDTAVYYCARQGTTALATRFFDVWGQGTLVTVSSGGGGSGGGGSGGGGSDIQMTQSPSSLSASVGDRVTITCKASQDVGTAVAWYQQKPGKAPKLLIYSASYRSTGVPSRFSGSGSGTDFTLTISSLQPEDFATYYCQHHYSAPWTFGGGTKVEIKESK

SEQ ID NO: 70 - DNA, 794 bp, Unknown
  IL13RA2 (HU07) VlVh scFv
atgcttctcctggtgacaagccttctgctctgtgagttaccacacccagcattcctcctgatcccagatattcagatgacccagagcccgagcagcctgagcgcgagcgtgggcgatcgcgtgaccattacctgcaccgcgagcctgagcgtgagcagcacctatctgcattggtatcagcagaaaccgggcaaagcgccgaaactgctgatttatagcaccagcaacctggcgagcggcgtgccgagccgctttagcggcagcggcagcggcaccgattttaccctgaccattagcagcctgcagccggaagattttgcgacctattattgccatcagtatcatcgcagcccgctgacctttggcggcggcaccaaagtggaaattaaaggtggtggtggttctggcggcggcggctccggtggtggtggttctgaagtgcagctggtggaaagcggcggcggcctggtgcagccgggcggcagcctgcgcctgagctgcgcggcgagcggctttacctttaccaaatatggcgtgcattgggtgcgccaggcgccgggcaaaggcctggaatgggtggcggtgaaatgggcgggcggcagcaccgattataacagcgcgctgatgagccgctttaccattagccgcgataacgcgaaaaacagcctgtatctgcagatgaacagcctgcgcgcggaagataccgcggtgtattattgcgcgcgcgatcatcgcgatgcgatggattattggggccagggcaccctggtgaccgtgagcagcgaatctaagta

SEQ ID NO: 71 - protein, 264 aa, Artificial Sequence
  IL13RA2 (HU07) VlVh scFv
MLLLVTSLLLCELPHPAFLLIPDIQMTQSPSSLSASVGDRVTITCTASLSVSSTYLHWYQQKPGKAPKLLIYSTSNLASGVPSRFSGSGSGTDFTLTISSLQPEDFATYYCHQYHRSPLTFGGGTKVEIKGGGGSGGGGSGGGGSEVQLVESGGGLVQPGGSLRLSCAASGFTFTKYGVHWVRQAPGKGLEWVAVKWAGGSTDYNSALMSRFTISRDNAKNSLYLQMNSLRAEDTAVYYCARDHRDAMDYWGQGTLVTVSSESK

SEQ ID NO: 72 - DNA, 794 bp, Unknown
  IL13RA2 (HU07) VlVh scFv
atgcttctcctggtgacaagccttctgctctgtgagttaccacacccagcattcctcctgatcccagaagtgcagctggtggaaagcggcggcggcctggtgcagccgggcggcagcctgcgcctgagctgcgcggcgagcggctttacctttaccaaatatggcgtgcattgggtgcgccaggcgccgggcaaaggcctggaatgggtggcggtgaaatgggcgggcggcagcaccgattataacagcgcgctgatgagccgctttaccattagccgcgataacgcgaaaaacagcctgtatctgcagatgaacagcctgcgcgcggaagataccgcggtgtattattgcgcgcgcgatcatcgcgatgcgatggattattggggccagggcaccctggtgaccgtgagcagcggtggtggtggttctggcggcggcggctccggtggtggtggttctgatattcagatgacccagagcccgagcagcctgagcgcgagcgtgggcgatcgcgtgaccattacctgcaccgcgagcctgagcgtgagcagcacctatctgcattggtatcagcagaaaccgggcaaagcgccgaaactgctgatttatagcaccagcaacctggcgagcggcgtgccgagccgctttagcggcagcggcagcggcaccgattttaccctgaccattagcagcctgcagccggaagattttgcgacctattattgccatcagtatcatcgcagcccgctgacctttggcggcggcaccaaagtggaaattaaagaatctaagta

SEQ ID NO: 73 - protein, 264 aa, Artificial Sequence
  IL13RA2 (HU07) VlVh
MLLLVTSLLLCELPHPAFLLIPEVQLVESGGGLVQPGGSLRLSCAASGFTFTKYGVHWVRQAPGKGLEWVAVKWAGGSTDYNSALMSRFTISRDNAKNSLYLQMNSLRAEDTAVYYCARDHRDAMDYWGQGTLVTVSSGGGGSGGGGSGGGGSDIQMTQSPSSLSASVGDRVTITCTASLSVSSTYLHWYQQKPGKAPKLLIYSTSNLASGVPSRFSGSGSGTDFTLTISSLQPEDFATYYCHQYHRSPLTFGGGTKVEIKESK

SEQ ID NO: 74 - DNA, 401 bp, Unknown
  Anti-IL13RA2 (IL13 ZETAKINE)
atgcttctcctggtgacaagccttctgctctgtgagttaccacacccagcattcctcctgatcccaggccctgtgcctccctctacagccctcaggtacctcattgaggagctggtcaacatcacccagaaccagaaggctccgctctgcaatggcagcatggtatggagcatcaacctgacagctggcatgtactgtgcagccctggaatccctgatcaacgtgtcaggctgcagtgccatcgagaagacccagaggatgctgagcggattctgcccgcacaaggtctcagctgggcagttttccagcttgcatgtccgagacaccaaaatcgaggtggcccagtttgtaaaggacctgctcttacatttaaagaaactttttcgcgagggacggttcaa

SEQ ID NO: 75 - protein, 133 aa, Artificial Sequence
  Anti-IL13RA2 (IL13 ZETAKINE) A
MLLLVTSLLLCELPHPAFLLIPGPVPPSTALRYLIEELVNITQNQKAPLCNGSMVWSINLTAGMYCAALESLINVSGCSAIEKTQRMLSGFCPHKVSAGQFSSLHVRDTKIEVAQFVKDLLLHLKKLFREGRF

SEQ ID NO: 76 - DNA, 807 bp, Unknown
  OAGD2 (8B6) VLVH SCFV NUCLEOTIDE SEQUENCE
atgcttctcctggtgacaagccttctgctctgtgagttaccacacccagcattcctcctgatcccagatgttgtgatgacccaaactccactctccctgcctgtcagtcttggagatcaagcctcaatctcttgcagatctagtcagagccttctaaaaaataatggaaacacctttttacattggtacctgcagaagtcaggccagtctccaaagctccttatctacaaagtttccaaccgactttctggggtcccagacaggttcagtggcagtggatcagggacatatttcacactcaagatcagcagagtggaggctgaggatctgggagtttatttctgctctcaaagtacacatattccgtacacattcggaggggggaccaagctcgagctgaaacgaggcggagggggctctggcggcggaggatctgggggagggggcagcgaggtgaaactggtggagtctggaggaggcttggtgctgcctggggattctctgagactctcctgtgcaacttctgagttcaccttcactgattactacatgacttgggtccgccagcctccaagaaaggcacttgagtggttgggttttattagaaacagagctaatggttacacaacagagtacaatccatctgtgaagggtcggttcaccatttccagagataattcccaaagcatcctctatcttcaaatgaacaccctgagaactgaggacagtgccacttattactgtgcaagagtctctaactgggcctttgactactggggccaaggcaccactctcacagtctcctca

SEQ ID NO: 77 - protein, 269 aa, Artificial Sequence
  OAGD2 (8B6) VlVh scFv
MLLLVTSLLLCELPHPAFLLIPDVVMTQTPLSLPVSLGDQASISCRSSQSLLKNNGNTFLHWYLQKSGQSPKLLIYKVSNRLSGVPDRFSGSGSGTYFTLKISRVEAEDLGVYFCSQSTHIPYTFGGGTKLELKRGGGGSGGGGSGGGGSEVKLVESGGGLVLPGDSLRLSCATSEFTFTDYYMTWVRQPPRKALEWLGFIRNRANGYTTEYNPSVKGRFTISRDNSQSILYLQMNTLRTEDSATYYCARVSNWAFDYWGQGTTLTVSS

SEQ ID NO: 78 - DNA, 810 bp, Unknown
  ROR1 (R12) scFv
atgctgctgctggtgacaagcctgctgctgtgcgagctgccccaccccgcctttctgctgatcccccaggaacagctcgtcgaaagcggcggcagactggtgacacctggcggcagcctgaccctgagctgcaaggccagcggcttcgacttcagcgcctactacatgagctgggtccgccaggcccctggcaagggactggaatggatcgccaccatctaccccagcagcggcaagacctactacgccacctgggtgaacggacggttcaccatctccagcgacaacgcccagaacaccgtggacctgcagatgaacagcctgacagccgccgaccgggccacctacttttgcgccagagacagctacgccgacgacggcgccctgttcaacatctggggccctggcaccctggtgacaatctctagcggcggaggcggatctggtggcggaggaagtggcggcggaggatctgagctggtgctgacccagagcccctctgtgtctgctgccctgggaagccctgccaagatcacctgtaccctgagcagcgcccacaagaccgacaccatcgactggtatcagcagctgcagggcgaggcccccagatacctgatgcaggtgcagagcgacggcagctacaccaagaggccaggcgtgcccgaccggttcagcggatctagctctggcgccgaccgctacctgatcatccccagcgtgcaggccgatgacgaggccgattactactgtggcgccgactacatcggcggctacgtgttcggcggaggcacccagctgaccgtgaccggc

SEQ ID NO: 79 - protein, 270 aa, Artificial Sequence
  ROR1 (R12) scFv
MLLLVTSLLLCELPHPAFLLIPQEQLVESGGRLVTPGGSLTLSCKASGFDFSAYYMSWVRQAPGKGLEWIATIYPSSGKTYYATWVNGRFTISSDNAQNTVDLQMNSLTAADRATYFCARDSYADDGALFNIWGPGTLVTISSGGGGSGGGGSGGGGSELVLTQSPSVSAALGSPAKITCTLSSAHKTDTIDWYQQLQGEAPRYLMQVQSDGSYTKRPGVPDRFSGSSSGADRYLIIPSVQADDEADYYCGADYIGGYVFGGGTQLTVTG

SEQ ID NO: 80 - DNA, 417 bp, Unknown
  CD33 (H2H12) VlVh scFv
atgcttctcctggtgacaagccttctgctctgtgagttaccacacccagcattcctcctgatcccacaggttcagctggtgcagtctggagctgaggtgaagaagcctggggcctcagtgaaggtctcctgcaaggcttctggttacacctttaccaattatgatataaattgggtgagacaggcccctggacaagggcttgagtggattggatggatttatcctggagatggtagtaccaaatataatgagaaattcaaggccaaggctaccctgacagctgacacatccaccagcacagcctacatggagctgaggagcctgagatctgatgacacagctgtgtattactgtgcttctggatatgaagatgctatggactactgggggcaagggaccacagtcacagtctcctca

SEQ ID NO: 81 - protein, 139 aa, Artificial Sequence
  CD33 (H2H12) VlVh scFv
MLLLVTSLLLCELPHPAFLLIPQVQLVQSGAEVKKPGASVKVSCKASGYTFTNYDINWVRQAPGQGLEWIGWIYPGDGSTKYNEKFKAKATLTADTSTSTAYMELRSLRSDDTAVYYCASGYEDAMDYWGQGTTVTVSS

SEQ ID NO: 82 - DNA, 387 bp, Unknown
  CD33 (H2H12) VlVh scFv
atgcttctcctggtgacaagccttctgctctgtgagttaccacacccagcattcctcctgatcccagacatccagatgacccagtctccatcctcactgtctgcatctgtaggagacagagtcaccatcaattgtaaggctagtcaggacattaatagctatttgagctggtttcagcagaaaccagggaaagcccctaagaccctgatctatagagcaaatagattggtagatggggtcccatcaaggttctctggcagtggatctgggcaagattatactctcaccatcagcagcctgcagcctgaagattttgcaacttattactgcttgcagtatgatgagtttcctctcacatttggaggagggaccaaggtggagatcaaa

SEQ ID NO: 83 - protein, 129 aa, Artificial Sequence
  CD33 (H2H12) VlVh scFv
MLLLVTSLLLCELPHPAFLLIPDIQMTQSPSSLSASVGDRVTINCKASQDINSYLSWFQQKPGKAPKTLIYRANRLVDGVPSRFSGSGSGQDYTLTISSLQPEDFATYYCLQYDEFPLTFGGGTKVEIK

SEQ ID NO: 84 - DNA, 450 bp, Unknown
  MESOTHELIN (P4) scFv
atgcttctcctggtgacaagccttctgctctgtgagttaccacacccagcattcctcctgatcccacaggtacagctgcagcagtcaggtccaggactcgtgacgccctcgcagaccctctcactcacctgtgccatctccggggacagtgtctctagcaacagtgctacttggaactggatcaggcagtccccatcgagaggccttgagtggctgggaaggacatactacaggtccaagtggtataacgactatgcagtatctgtgaaaagtcgaatgagcatcaacccagacacatccaagaaccagttctccctgcagctgaactctgtgactcccgaggacacggctgtgtattactgtgcaagaggaatgatgacttactattacggtatggacgtctggggccaagggaccacggtcaccgtctcctcaggaattctaggatcc

SEQ ID NO: 85 - protein, 150 aa, Artificial Sequence
  MESOTHELIN (P4) scFv
MLLLVTSLLLCELPHPAFLLIPQVQLQQSGPGLVTPSQTLSLTCAISGDSVSSNSATWNWIRQSPSRGLEWLGRTYYRSKWYNDYAVSVKSRMSINPDTSKNQFSLQLNSVTPEDTAVYYCARGMMTYYYGMDVWGQGTTVTVSSGILGS

SEQ ID NO: 86 - DNA, 1344 bp, Unknown
  VAR2CSA (ID1-DBL2XB) scFv
atgcttctcctggtgacaagccttctgctctgtgagttaccacacccagcattcctcctgatcccaagtctcacgaatgggtataagtgcgacaaatgcaaatcaggcacatcccggtccaaaaaaaaatggatctggaaaaagagcagcgggaatgaggagggcctgcaggaagaatacgctaacacaatcggactgccccctcgaactcaatctctgtaccttgggaacttgcctaaactggaaaacgtctgtgaagacgtcaaggacataaacttcgatacgaaagagaagttcctggctggatgccttatcgtgagctttcacgagggaaagaatctgaagaaaaggtacccacagaataaaaactctggcaataaagagaatttgtgcaaggccctggagtactcttttgcggactatggcgatctcataaagggcacaagcatctgggataatgagtataccaaggatctggagctgaatctgcagaataactttgggaaattgtttgggaagtatattaaaaaaaataataccgccgagcaggacacatcctactcttccctcgacgagctgcgggagtcatggtggaacaccaacaaaaagtatatctggacggcaatgaaacatggcgcggaaatgaatatcaccacttgtaatgcagacggctctgtcaccgggtccggttcttcttgcgatgatataccaaccatcgatttgattccgcagtatctgagatttctccaagagtgggtggaaaatttttgcgagcagaggcaagctaaggtcaaggacgtgatcaccaattgtaaaagttgcaaagaatcagggaacaagtgcaaaaccgagtgtaagacgaagtgcaaggacgaatgcgagaaatataaaaaattcatcgaggcttgtggaacagccgggggtgggattgggaccgcaggcagcccatggagcaagcggtgggaccaaatctataaacgatacagcaagcacatcgaagatgccaagcggaaccgcaaagctggcacaaaaaactgtgggactagcagcacgactaatgccgcggcaagcactgatgaaaataaatgcgtgcaaagtgacatcgactctttcttcaaacacctgatcgatatcggtcttactacgccaagcagctacctcagtaatgttctggatgataatatttgtggggcggacaaagcaccttggactacctacaccacctataccacaacagagaagtgtaataaagagagagacaaatcaaagtctcagagctctgatacactggtcgttgtgaatgtgccaagccctttggggaatacgccctacagatataaatac

SEQ ID NO: 87 - protein, 448 aa, Artificial Sequence
  VAR2CSA (ID1-DBL2XB) scFv
MLLLVTSLLLCELPHPAFLLIPSLTNGYKCDKCKSGTSRSKKKWIWKKSSGNEEGLQEEYANTIGLPPRTQSLYLGNLPKLENVCEDVKDINFDTKEKFLAGCLIVSFHEGKNLKKRYPQNKNSGNKENLCKALEYSFADYGDLIKGTSIWDNEYTKDLELNLQNNFGKLFGKYIKKNNTAEQDTSYSSLDELRESWWNTNKKYIWTAMKHGAEMNITTCNADGSVTGSGSSCDDIPTIDLIPQYLRFLQEWVENFCEQRQAKVKDVITNCKSCKESGNKCKTECKTKCKDECEKYKKFIEACGTAGGGIGTAGSPWSKRWDQIYKRYSKHIEDAKRNRKAGTKNCGTSSTTNAAASTDENKCVQSDIDSFFKHLIDIGLTTPSSYLSNVLDDNICGADKAPWTTYTTYTTTEKCNKERDKSKSQSSDTLVVVNVPSPLGNTPYRYKY

SEQ ID NO: 88 - DNA, 2202 bp, Unknown
  CCR(CD122)
atgcttctcctggtgacaagccttctgctctgtgagttaccacacccagcattcctcctgatcccagattgtgatattgaaggtaaagatggcaaacaatatgagagtgttctaatggtcagcatcgatcaattattggacagcatgaaagaaattggtagcaattgcctgaataatgaatttaacttttttaaaagacatatctgtgatgctaataaggaaggtatgtttttattccgtgctgctcgcaagttgaggcaatttcttaaaatgaatagcactggtgattttgatctccacttattaaaagtttcagaaggcacaacaatactgttgaactgcactggccaggttaaaggaagaaaaccagctgccctgggtgaagcccaaccaacaaagagtttggaagaaaataaatctttaaaggaacagaaaaaactgaatgacttgtgtttcctaaagagactattacaagagataaaaacttgttggaataaaattttgatgggcactaaagaacacggaggcggtgggagcggaggcggtgggagcatgacaattctaggtacaacttttggcatggttttttctttacttcaagtcgtttctggagaaagtggctatgctcaaaatggagacttggaagatgcagaactggatgactactcattctcatgctatagccagttggaagtgaatggatcgcagcactcactgacctgtgcttttgaggacccagatgtcaacatcaccaatctggaatttgaaatatgtggggccctcgtggaggtaaagtgcctgaatttcaggaaactacaagagatatatttcatcgagacaaagaaattcttactgattggaaagagcaatatatgtgtgaaggttggagaaaagagtctaacctgcaaaaaaatagacctaaccactatagttaaacctgaggctccttttgacctgagtgtcatctatcgggaaggagccaatgactttgtggtgacatttaatacatcacacttgcaaaagaagtatgtaaaagttttaatgcacgatgtagcttaccgccaggaaaaggatgaaaacaaatggacgcatgtgaatttatccagcacaaaactgacactcctgcagagaaagctccaaccggcagcaatgtatgagattaaagttcgatccatccctgatcactattttaaaggcttctggagtgaatggagtccaagttattacttcagaactccagagatcaataatagctcaggggagatggatcctatcttactaaccatcagcattttgagttttttctctgtcgctctgttggtcatcttggcctgtgtgttatggaactgcaggaacaccgggccatggctgaagaaggtcctgaagtgtaacaccccagacccctcgaagttcttttcccagctgagctcagagcatggaggagacgtccagaagtggctctcttcgcccttcccctcatcgtccttcagccctggcggcctggcacctgagatctcgccactagaagtgctggagagggacaaggtgacgcagctgctcctgcagcaggacaaggtgcctgagcccgcatccttaagcagcaaccactcgctgaccagctgcttcaccaaccagggttacttcttcttccacctcccggatgccttggagatagaggcctgccaggtgtactttacttacgacccctactcagaggaagaccctgatgagggtgtggccggggcacccacagggtcttccccccaacccctgcagcctctgtcaggggaggacgacgcctactgcaccttcccctccagggatgacctgctgctcttctcccccagtctcctcggtggccccagccccccaagcactgcccctgggggcagtggggccggtgaagagaggatgcccccttctttgcaagaaagagtccccagagactgggacccccagcccctggggcctcccaccccaggagtcccagacctggtggattttcagccaccccctgagctggtgctgcgagaggctggggaggaggtccctgacgctggccccagggagggagtcagtttcccctggtccaggcctcctgggcagggggagttcagggcccttaatgctcgcctgcccctgaacactgatgcctacttgtccctccaagaactccagggtcaggacccaactcacttggtg

SEQ ID NO: 89 - protein, 734 aa, Artificial Sequence
  CCR(CD122)
MLLLVTSLLLCELPHPAFLLIPDCDIEGKDGKQYESVLMVSIDQLLDSMKEIGSNCLNNEFNFFKRHICDANKEGMFLFRAARKLRQFLKMNSTGDFDLHLLKVSEGTTILLNCTGQVKGRKPAALGEAQPTKSLEENKSLKEQKKLNDLCFLKRLLQEIKTCWNKILMGTKEHGGGGSGGGGSMTILGTTFGMVFSLLQVVSGESGYAQNGDLEDAELDDYSFSCYSQLEVNGSQHSLTCAFEDPDVNITNLEFEICGALVEVKCLNFRKLQEIYFIETKKFLLIGKSNICVKVGEKSLTCKKIDLTTIVKPEAPFDLSVIYREGANDFVVTFNTSHLQKKYVKVLMHDVAYRQEKDENKWTHVNLSSTKLTLLQRKLQPAAMYEIKVRSIPDHYFKGFWSEWSPSYYFRTPEINNSSGEMDPILLTISILSFFSVALLVILACVLWNCRNTGPWLKKVLKCNTPDPSKFFSQLSSEHGGDVQKWLSSPFPSSSFSPGGLAPEISPLEVLERDKVTQLLLQQDKVPEPASLSSNHSLTSCFTNQGYFFFHLPDALEIEACQVYFTYDPYSEEDPDEGVAGAPTGSSPQPLQPLSGEDDAYCTFPSRDDLLLFSPSLLGGPSPPSTAPGGSGAGEERMPPSLQERVPRDWDPQPLGPPTPGVPDLVDFQPPPELVLREAGEEVPDAGPREGVSFPWSRPPGQGEFRALNARLPLNTDAYLSLQELQGQDPTHLV

SEQ ID NO: 90 - DNA, 1014 bp, Unknown
  PD1ECD-IFNALPHA
atgcagatccctcaggccccttggcctgtcgtgtgggctgtgctgcagctgggatggcggcctggctggtttctggacagccccgacagaccctggaacccccctacattttcccctgccctgctggtcgtgaccgagggcgacaatgccaccttcacctgtagcttcagcaacaccagcgagagcttcgtgctgaactggtacagaatgagccccagcaaccagaccgacaagctggccgccttccccgaggatagatctcagcccggccaggactgccggttcagagtgacccagctgcccaacggccgggacttccacatgtctgtcgtgcgggccagacggaacgacagcggcacatatctgtgcggcgccatcagcctggcccccaaggcccagatcaaagagagcctgagagccgagctgagagtgaccgagagaagggccgaagtgcctaccgcccaccctagcccatctccaagacctgccggccagttccagacactcgtgggcggaggatgcgacctgcctcagacacacagcctgggcagcagacggaccctgatgctgctggcccagatgcggaagatcagcctgttcagctgcctgaaggaccggcacgacttcggcttccctcaggaagagttcggcaaccagtttcagaaggccgagacaatccccgtgctgcacgagatgatccagcagatcttcaacctgttctccaccaaggacagcagcgccgcctgggacgagacactgctggacaagttctacaccgagctgtaccagcagctgaatgacctggaagcctgcgtgatccagggcgtgggcgtgacagagacacccctgatgaaggaagatagcatcctggccgtgcgcaagtacttccagcggatcaccctgtacctgaaagagaagaagtacagcccctgcgcctgggaggtcgtgcgcgccgagatcatgagaagcttcagcctgagcaccaacctgcaggaaagcctgcggagcaaagaa

SEQ ID NO: 91 - protein, 338 aa, Artificial Sequence
  PD1ECD-IFNALPHA
MQIPQAPWPVVWAVLQLGWRPGWFLDSPDRPWNPPTFSPALLVVTEGDNATFTCSFSNTSESFVLNWYRMSPSNQTDKLAAFPEDRSQPGQDCRFRVTQLPNGRDFHMSVVRARRNDSGTYLCGAISLAPKAQIKESLRAELRVTERRAEVPTAHPSPSPRPAGQFQTLVGGGCDLPQTHSLGSRRTLMLLAQMRKISLFSCLKDRHDFGFPQEEFGNQFQKAETIPVLHEMIQQIFNLFSTKDSSAAWDETLLDKFYTELYQQLNDLEACVIQGVGVTETPLMKEDSILAVRKYFQRITLYLKEKKYSPCAWEVVRAEIMRSFSLSTNLQESLRSKE

SEQ ID NO: 92 - DNA, 2382 bp, Unknown
  STAT5A
atggcgggctggatccaggcccagcagctgcagggagacgcgctgcgccagatgcaggtgctgtacggccagcacttccccatcgaggtccggcactacttggcccagtggattgagagccagccatgggatgccattgacttggacaatccccaggacagagcccaagccacccagctcctggagggcctggtgcaggagctgcagaagaaggcggagcaccaggtgggggaagatgggtttttactgaagatcaagctggggcactacgccacgcagctccagaaaacatatgaccgctgccccctggagctggtccgctgcatccggcacattctgtacaatgaacagaggctggtccgagaagccaacaattgcagctctccggctgggatcctggttgacgccatgtcccagaagcaccttcagatcaaccagacatttgaggagctgcgactggtcacgcaggacacagagaatgagctgaagaaactgcagcagactcaggagtacttcatcatccagtaccaggagagcctgaggatccaagctcagtttgcccagctggcccagctgagcccccaggagcgtctgagccgggagacggccctccagcagaagcaggtgtctctggaggcctggttgcagcgtgaggcacagacactgcagcagtaccgcgtggagctggccgagaagcaccagaagaccctgcagctgctgcggaagcagcagaccatcatcctggatgacgagctgatccagtggaagcggcggcagcagctggccgggaacggcgggccccccgagggcagcctggacgtgctacagtcctggtgtgagaagttggccgagatcatctggcagaaccggcagcagatccgcagggctgagcacctctgccagcagctgcccatccccggcccagtggaggagatgctggccgaggtcaacgccaccatcacggacattatctcagccctggtgaccagcacattcatcattgagaagcagcctcctcaggtcctgaagacccagaccaagtttgcagccaccgtacgcctgctggtgggcgggaagctgaacgtgcacatgaatcccccccaggtgaaggccaccatcatcagtgagcagcaggccaagtctctgcttaaaaatgagaacacccgcaacgagtgcagtggtgagatcctgaacaactgctgcgtgatggagtaccaccaagccacgggcaccctcagtgcccacttcaggaacatgtcactgaagaggatcaagcgtgctgaccggcggggtgcagagtccgtgacagaggagaagttcacagtcctgtttgagtctcagttcagtgttggcagcaatgagcttgtgttccaggtgaagactctgtccctacctgtggttgtcatcgtccacggcagccaggaccacaatgccacggctactgtgctgtgggacaatgcctttgctgagccgggcagggtgccatttgccgtgcctgacaaagtgctgtggccgcagctgtgtgaggcgctcaacatgaaattcaaggccgaagtgcagagcaaccggggcctgaccaaggagaacctcgtgttcctggcgcagaaactgttcaacaacagcagcagccacctggaggactacagtggcctgtccgtgtcctggtcccagttcaacagggagaacttgccgggctggaactacaccttctggcagtggtttgacggggtgatggaggtgttgaagaagcaccacaagccccactggaatgatggggccatcctaggttttgtgaataagcaacaggcccacgacctgctcatcaacaagcccgacgggaccttcttgttgcgctttagtgactcagaaatcgggggcatcaccatcgcctggaagtttgattccccggaacgcaacctgtggaacctgaaaccattcaccacgcgggatttctccatcaggtccctggctgaccggctgggggacctgagctatctcatctatgtgtttcctgaccgccccaaggatgaggtcttctccaagtactacactcctgtgctggctaaagctgttgatggatatgtgaaaccacagatcaagcaagtggtccctgagtttgtgaatgcatctgcagatgctgggggcagcagcgccacgtacatggaccaggccccctccccagctgtgtgcccccaggctccctataacatgtacccacagaaccctgaccatgtactcgatcaggatggagaattcgacctggatgagaccatggatgtggccaggcacgtggaggaactcttacgccgaccaatggacagtcttgactcccgcctctcgccccctgccggtcttttcacctctgccagaggctccctctca

SEQ ID NO: 93 - protein, 794 aa, Artificial Sequence
  STAT5A
MAGWIQAQQLQGDALRQMQVLYGQHFPIEVRHYLAQWIESQPWDAIDLDNPQDRAQATQLLEGLVQELQKKAEHQVGEDGFLLKIKLGHYATQLQKTYDRCPLELVRCIRHILYNEQRLVREANNCSSPAGILVDAMSQKHLQINQTFEELRLVTQDTENELKKLQQTQEYFIIQYQESLRIQAQFAQLAQLSPQERLSRETALQQKQVSLEAWLQREAQTLQQYRVELAEKHQKTLQLLRKQQTIILDDELIQWKRRQQLAGNGGPPEGSLDVLQSWCEKLAEIIWQNRQQIRRAEHLCQQLPIPGPVEEMLAEVNATITDIISALVTSTFIIEKQPPQVLKTQTKFAATVRLLVGGKLNVHMNPPQVKATIISEQQAKSLLKNENTRNECSGEILNNCCVMEYHQATGTLSAHFRNMSLKRIKRADRRGAESVTEEKFTVLFESQFSVGSNELVFQVKTLSLPVVVIVHGSQDHNATATVLWDNAFAEPGRVPFAVPDKVLWPQLCEALNMKFKAEVQSNRGLTKENLVFLAQKLFNNSSSHLEDYSGLSVSWSQFNRENLPGWNYTFWQWFDGVMEVLKKHHKPHWNDGAILGFVNKQQAHDLLINKPDGTFLLRFSDSEIGGITIAWKFDSPERNLWNLKPFTTRDFSIRSLADRLGDLSYLIYVFPDRPKDEVFSKYYTPVLAKAVDGYVKPQIKQVVPEFVNASADAGGSSATYMDQAPSPAVCPQAPYNMYPQNPDHVLDQDGEFDLDETMDVARHVEELLRRPMDSLDSRLSPPAGLFTSARGSLS

SEQ ID NO: 94 - DNA, 2382 bp, Unknown
  constitutively active-STAT5A
atggcgggctggatccaggcccagcagctgcagggagacgcgctgcgccagatgcaggtgctgtacggccagcacttccccatcgaggtccggcactacttggcccagtggattgagagccagccatgggatgccattgacttggacaatccccaggacagagcccaagccacccagctcctggagggcctggtgcaggagctgcagaagaaggcggagcaccaggtgggggaagatgggtttttactgaagatcaagctggggcactacgccacgcagctccagaaaacatatgaccgctgccccctggagctggtccgctgcatccggcacattctgtacaatgaacagaggctggtccgagaagccaacaattgcagctctccggctgggatcctggttgacgccatgtcccagaagcaccttcagatcaaccagacatttgaggagctgcgactggtcacgcaggacacagagaatgagctgaagaaactgcagcagactcaggagtacttcatcatccagtaccaggagagcctgaggatccaagctcagtttgcccagctggcccagctgagcccccaggagcgtctgagccgggagacggccctccagcagaagcaggtgtctctggaggcctggttgcagcgtgaggcacagacactgcagcagtaccgcgtggagctggccgagaagcaccagaagaccctgcagctgctgcggaagcagcagaccatcatcctggatgacgagctgatccagtggaagcggcggcagcagctggccgggaacggcgggccccccgagggcagcctggacgtgctacagtcctggtgtgagaagttggccgagatcatctggcagaaccggcagcagatccgcagggctgagcgcctctgccagcagctgcccatccccggcccagtggaggagatgctggccgaggtcaacgccaccatcacggacattatctcagccctggtgaccagcacattcatcattgagaagcagcctcctcaggtcctgaagacccagaccaagtttgcagccaccgtacgcctgctggtgggcgggaagctgaacgtgcacatgaatcccccccaggtgaaggccaccatcatcagtgagcagcaggccaagtctctgcttaaaaatgagaacacccgcaacgagtgcagtggtgagatcctgaacaactgctgcgtgatggagtaccaccaagccacgggcaccctcagtgcccacttcaggaacatgtcactgaagaggatcaagcgtgctgaccggcggggtgcagagtccgtgacagaggagaagttcacagtcctgtttgagtctcagttcagtgttggcagcaatgagcttgtgttccaggtgaagactctgtccctacctgtggttgtcatcgtccacggcagccaggaccacaatgccacggctactgtgctgtgggacaatgcctttgctgagccgggcagggtgccatttgccgtgcctgacaaagtgctgtggccgcagctgtgtgaggcgctcaacatgaaattcaaggccgaagtgcagagcaaccggggcctgaccaaggagaacctcgtgttcctggcgcagaaactgttcaacaacagcagcagccacctggaggactacagtggcctgtccgtgtcctggtcccagttcaacagggagaacttgccgggctggaactacaccttctggcagtggtttgacggggtgatggaggtgttgaagaagcaccacaagccccactggaatgatggggccatcctaggttttgtgaataagcaacaggcccacgacctgctcatcaacaagcccgacgggaccttcttgttgcgctttagtgactcagaaatcgggggcatcaccatcgcctggaagtttgattccccggaacgcaacctgtggaacctgaaaccattcaccacgcgggatttctccatcaggtccctggctgaccggctgggggacctgagctatctcatctatgtgtttcctgaccgccccaaggatgaggtcttctccaagtactacactcctgtgctggctaaagctgttgatggatatgtgaaaccacagatcaagcaagtggtccctgagtttgtgaatgcatttgcagatgctgggggcagcagcgccacgtacatggaccaggccccctccccagctgtgtgcccccaggctccctataacatgtacccacagaaccctgaccatgtactcgatcaggatggagaattcgacctggatgagaccatggatgtggccaggcacgtggaggaactcttacgccgaccaatggacagtcttgactcccgcctctcgccccctgccggtcttttcacctctgccagaggctccctctca

SEQ ID NO: 95 - protein, 794 aa, Artificial Sequence
  constitutively active-STAT5A
  constitutively active-STAT5A
MAGWIQAQQLQGDALRQMQVLYGQHFPIEVRHYLAQWIESQPWDAIDLDNPQDRAQATQLLEGLVQELQKKAEHQVGEDGFLLKIKLGHYATQLQKTYDRCPLELVRCIRHILYNEQRLVREANNCSSPAGILVDAMSQKHLQINQTFEELRLVTQDTENELKKLQQTQEYFIIQYQESLRIQAQFAQLAQLSPQERLSRETALQQKQVSLEAWLQREAQTLQQYRVELAEKHQKTLQLLRKQQTIILDDELIQWKRRQQLAGNGGPPEGSLDVLQSWCEKLAEIIWQNRQQIRRAERLCQQLPIPGPVEEMLAEVNATITDIISALVTSTFIIEKQPPQVLKTQTKFAATVRLLVGGKLNVHMNPPQVKATIISEQQAKSLLKNENTRNECSGEILNNCCVMEYHQATGTLSAHFRNMSLKRIKRADRRGAESVTEEKFTVLFESQFSVGSNELVFQVKTLSLPVVVIVHGSQDHNATATVLWDNAFAEPGRVPFAVPDKVLWPQLCEALNMKFKAEVQSNRGLTKENLVFLAQKLFNNSSSHLEDYSGLSVSWSQFNRENLPGWNYTFWQWFDGVMEVLKKHHKPHWNDGAILGFVNKQQAHDLLINKPDGTFLLRFSDSEIGGITIAWKFDSPERNLWNLKPFTTRDFSIRSLADRLGDLSYLIYVFPDRPKDEVFSKYYTPVLAKAVDGYVKPQIKQVVPEFVNAFADAGGSSATYMDQAPSPAVCPQAPYNMYPQNPDHVLDQDGEFDLDETMDVARHVEELLRRPMDSLDSRLSPPAGLFTSARGSLS

SEQ ID NO: 96 - DNA, 837 bp, Unknown
  dominant negative TGFB-RII
atgggtcgggggctgctcaggggcctgtggccgctgcacatcgtcctgtggacgcgtatcgccagcacgatcccaccgcacgttcagaagtcggttaataacgacatgatagtcactgacaacaacggtgcagtcaagtttccacaactgtgtaaattttgtgatgtgagattttccacctgtgacaaccagaaatcctgcatgagcaactgcagcatcacctccatctgtgagaagccacaggaagtctgtgtggctgtatggagaaagaatgacgagaacataacactagagacagtttgccatgaccccaagctcccctaccatgactttattctggaagatgctgcttctccaaagtgcattatgaaggaaaaaaaaaagcctggtgagactttcttcatgtgttcctgtagctctgatgagtgcaatgacaacatcatcttctcagaagaatataacaccagcaatcctgacttgttgctagtcatatttcaagtgacaggcatcagcctcctgccaccactgggagttgccatatctgtcatcatcatcttctactgctaccgcgttaaccggcagcagaagctgagttcaacctgggaaaccggcaagacgcggaagctcatggagttcagcgagcactgtgccatcatcctggaagatgaccgctctgacatcagctccacgtgtgccaacaacatcaaccacaacacagagctgctgcccattgagctggacaccctggtggggaaaggtcgctttgctgaggtctataaggccaagctgaagcagaacacttcagagcagtttgagacagtggcagtcaagatcttt

SEQ ID NO: 97 - protein, 279 aa, Artificial Sequence
  dominant negative TGFBRII
MGRGLLRGLWPLHIVLWTRIASTIPPHVQKSVNNDMIVTDNNGAVKFPQLCKFCDVRFSTCDNQKSCMSNCSITSICEKPQEVCVAVWRKNDENITLETVCHDPKLPYHDFILEDAASPKCIMKEKKKPGETFFMCSCSSDECNDNIIFSEEYNTSNPDLLLVIFQVTGISLLPPLGVAISVIIIFYCYRVNRQQKLSSTWETGKTRKLMEFSEHCAIILEDDRSDISSTCANNINHNTELLPIELDTLVGKGRFAEVYKAKLKQNTSEQFETVAVKIF

SEQ ID NO: 98 - DNA, 1788 bp, Unknown
  dominant negative SHP1
atggtgaggtggtttcaccgagacctcagtgggctggatgcagagaccctgctcaagggccgaggtgtccacggtagcttcctggctcggcccagtcgcaagaaccagggtgacttctcgctctccgtcagggtgggggatcaggtgacccatattcggatccagaactcaggggatttctatgacctgtatggaggggagaagtttgcgactctgacagagctggtggagtactacactcagcagcagggtgtcctgcaggaccgcgacggcaccatcatccacctcaagtacccgctgaactgctccgatcccactagtgagaggtggtaccatggccacatgtctggcgggcaggcagagacgctgctgcaggccaagggcgagccctggacgtttcttgtgcgtgagagcctcagccagcctggagacttcgtgctttctgtgctcagtgaccagcccaaggctggcccaggctccccgctcagggtcacccacatcaaggtcatgtgcgagggtggacgctacacagtgggtggtttggagaccttcgacagcctcacggacctggtggagcatttcaagaagacggggattgaggaggcctcaggcgcctttgtctacctgcggcagccgtactatgccacgagggtgaatgcggctgacattgagaaccgagtgttggaactgaacaagaagcaggagtccgaggatacagccaaggctggcttctgggaggagtttgagagtttgcagaagcaggaggtgaagaacttgcaccagcgtctggaagggcagcggccagagaacaagggcaagaaccgctacaagaacattctcccctttgaccacagccgagtgatcctgcagggacgggacagtaacatccccgggtccgactacatcaatgccaactacatcaagaaccagctgctaggccctgatgagaacgctaagacctacatcgccagccagggctgtctggaggccacggtcaatgacttctggcagatggcgtggcaggagaacagccgtgtcatcgtcatgaccacccgagaggtggagaaaggccggaacaaatgcgtcccatactggcccgaggtgggcatgcagcgtgcttatgggccctactctgtgaccaactgcggggagcatgacacaaccgaatacaaactccgtaccttacaggtctccccgctggacaatggagacctgattcgggagatctggcattaccagtacctgagctggcccgaccatggggtccccagtgagcctgggggtgtcctcagcttcctggaccagatcaaccagcggcaggaaagtctgcctcacgcagggcccatcatcgtgcactccagcgccggcatcggccgcacaggcaccatcattgtcatcgacatgctcatggagaacatctccaccaagggcctggactgtgacattgacatccagaagaccatccagatggtgcgggcgcagcgctcgggcatggtgcagacggaggcgcagtacaagttcatctacgtggccatcgcccagttcattgaaaccactaagaagaagctggaggtcctgcagtcgcagaagggccaggagtcggagtacgggaacatcacctatcccccagccatgaagaatgcccatgccaaggcctcccgcacctcgtccaaacacaaggaggatgtgtatgagaacctgcacactaagaacaagagggaggagaaagtgaagaagcagcggtcagcagacaaggagaagagcaagggttccctcaagaggaagtga

SEQ ID NO: 99 - protein, 595 aa, Artificial Sequence
  dominant negative SHP1
MVRWFHRDLSGLDAETLLKGRGVHGSFLARPSRKNQGDFSLSVRVGDQVTHIRIQNSGDFYDLYGGEKFATLTELVEYYTQQQGVLQDRDGTIIHLKYPLNCSDPTSERWYHGHMSGGQAETLLQAKGEPWTFLVRESLSQPGDFVLSVLSDQPKAGPGSPLRVTHIKVMCEGGRYTVGGLETFDSLTDLVEHFKKTGIEEASGAFVYLRQPYYATRVNAADIENRVLELNKKQESEDTAKAGFWEEFESLQKQEVKNLHQRLEGQRPENKGKNRYKNILPFDHSRVILQGRDSNIPGSDYINANYIKNQLLGPDENAKTYIASQGCLEATVNDFWQMAWQENSRVIVMTTREVEKGRNKCVPYWPEVGMQRAYGPYSVTNCGEHDTTEYKLRTLQVSPLDNGDLIREIWHYQYLSWPDHGVPSEPGGVLSFLDQINQRQESLPHAGPIIVHSSAGIGRTGTIIVIDMLMENISTKGLDCDIDIQKTIQMVRAQRSGMVQTEAQYKFIYVAIAQFIETTKKKLEVLQSQKGQESEYGNITYPPAMKNAHAKASRTSSKHKEDVYENLHTKNKREEKVKKQRSADKEKSKGSLKRK

SEQ ID NO: 100 - DNA, 1035 bp, Unknown
  PD1TM-MYD88
atgcttctcctggtgacaagccttctgctctgtgagttaccacacccagcattcctcctgatcccaggcggaggagtgggagtcgtgggcggactgctgggatctctggtgctgctcgtgtgggtgctggccgtgattggcggaggaatggctgctggcggacctggcgctggatctgctgctcctgtgtctagcaccagcagcctgcctctggccgccctgaatatgagagtgcggcggagactgagcctgttcctgaacgtgcggacacaggtggccgccgattggacagctctggccgaggaaatggacttcgagtacctggaaatccggcagctggaaacccaggccgaccctacaggacgcctgctggatgcttggcagggcagaccaggcgcttctgtggggagactgctggaactgctgaccaagctgggccgggacgacgtgctgctggaactgggccctagcatcgaagaggactgccagaagtacatcctgaagcagcagcaggaagaggccgagaagcctctgcaggtggcagccgtggatagcagcgtgccaagaacagctgagctggccggaatcaccaccctggacgatcctctgggccacatgcccgagagattcgacgccttcatctgctactgccccagcgacatccagttcgtgcaggaaatgatcagacagctggaacagaccaactaccggctgaagctgtgcgtgtccgaccgggatgtgctgcctggcacctgtgtgtggtctatcgccagcgagctgatcgagaagcggtgcagacggatggtcgtggtggtgtccgacgactacctgcagtccaaagagtgcgacttccagaccaagttcgccctgagcctgagccctggcgcccaccagaagagactgatccccatcaagtacaaggccatgaagaaagagttccccagcatcctgcggttcatcaccgtgtgcgactacaccaacccctgcaccaagtcctggttctggaccagactggccaaggccctgtctctgcct

SEQ ID NO: 101 - protein, 345 aa, Artificial Sequence
  PD1TM-MYD88
MLLLVTSLLLCELPHPAFLLIPGGGVGVVGGLLGSLVLLVWVLAVIGGGMAAGGPGAGSAAPVSSTSSLPLAALNMRVRRRLSLFLNVRTQVAADWTALAEEMDFEYLEIRQLETQADPTGRLLDAWQGRPGASVGRLLELLTKLGRDDVLLELGPSIEEDCQKYILKQQQEEAEKPLQVAAVDSSVPRTAELAGITTLDDPLGHMPERFDAFICYCPSDIQFVQEMIRQLEQTNYRLKLCVSDRDVLPGTCVWSIASELIEKRCRRMVVVVSDDYLQSKECDFQTKFALSLSPGAHQKRLIPIKYKAMKKEFPSILRFITVCDYTNPCTKSWFWTRLAKALSLP

SEQ ID NO: 102 - DNA, 36 bp, Unknown
  IGG4 HINGE
gagagcaagtacggaccgccctgccccccttgccct

SEQ ID NO: 103 - protein, 12 aa, Artificial Sequence
  IGG4 HINGE
ESKYGPPCPPCP

SEQ ID NO: 104 - DNA, 330 bp, Unknown
  IGG4-CH2(L235D, N297Q)
gcccccgagttcgacggcggacccagcgtgttcctgttcccccccaagcccaaggacaccctgatgatcagccggacccccgaggtgacctgcgtggtggtggacgtgagccaggaagatcccgaggtccagttcaattggtacgtggacggcgtggaagtgcacaacgccaagaccaagcccagagaggaacagttccagagcacctaccgggtggtgtctgtgctgaccgtgctgcaccaggactggctgaacggcaaagaatacaagtgcaaggtgtccaacaagggcctgcccagcagcatcgaaaagaccatcagcaaggccaag

SEQ ID NO: 105 - protein, 110 aa, Artificial Sequence
  IGG4-CH2(L235D, N297Q)
APEFDGGPSVFLFPPKPKDTLMISRTPEVTCVVVDVSQEDPEVQFNWYVDGVEVHNAKTKPREEQFQSTYRVVSVLTVLHQDWLNGKEYKCKVSNKGLPSSIEKTISKAK

SEQ ID NO: 106 - DNA, 321 bp, Unknown
  IGG4-CH3
ggccagcctcgcgagccccaggtgtacaccctgcctccctcccaggaagagatgaccaagaaccaggtgtccctgacctgcctggtgaagggcttctaccccagcgacatcgccgtggagtgggagagcaacggccagcctgagaacaactacaagaccacccctcccgtgctggacagcgacggcagcttcttcctgtacagccggctgaccgtggacaagagccggtggcaggaaggcaacgtctttagctgcagcgtgatgcacgaggccctgcacaaccactacacccagaagagcctgagcctgtccctgggcaag

SEQ ID NO: 107 - protein, 107 aa, Artificial Sequence
  IGG4-CH3
GQPREPQVYTLPPSQEEMTKNQVSLTCLVKGFYPSDIAVEWESNGQPENNYKTTPPVLDSDGSFFLYSRLTVDKSRWQEGNVFSCSVMHEALHNHYTQKSLSLSLGK

SEQ ID NO: 108 - DNA, 225 bp, Unknown
  CD8 hinge/transmembrane domain
gaatctaagtacggaccggccaagcctaccaccacccctgcccctagacctccaacacccgccccaacaatcgccagccagcctctgtctctgaggcccgaggcttgtagaccagctgctggcggagccgtgcacaccagaggactggatttcgcctgcgacatctacatctgggcccctctggccggcacatgtggcgtgctgctgctgagcctcgtgatcacc

SEQ ID NO: 109 - protein, 75 aa, Artificial Sequence
  CD8 hinge/transmembrane domain
ESKYGPAKPTTTPAPRPPTPAPTIASQPLSLRPEACRPAAGGAVHTRGLDFACDIYIWAPLAGTCGVLLLSLVIT

SEQ ID NO: 110 - DNA, 84 bp, Unknown
  CD28 transmembrane domain
atgttctgggtgctggtggtggtcggaggcgtgctggcctgctacagcctgctggtcaccgtggccttcatcatcttttgggtg

SEQ ID NO: 111 - protein, 28 aa, Artificial Sequence
  CD28 transmembrane domain
MFWVLVVVGGVLACYSLLVTVAFIIFWV

SEQ ID NO: 112 - DNA, 225 bp, Unknown; identical to SEQ ID NO: 108
  CD8 hinge/ transmembrane domain

SEQ ID NO: 113 - protein, 75 aa, Artificial Sequence; identical to SEQ ID NO: 109
  CD8 hinge/ transmembrane domain

SEQ ID NO: 114 - DNA, 336 bp, Unknown
  CD3 Zeta
cgggtgaagttcagcagaagcgccgacgcccctgcctaccagcagggccagaatcagctgtacaacgagctgaacctgggcagaagggaagagtacgacgtcctggataagcggagaggccgggaccctgagatgggcggcaagcctcggcggaagaacccccaggaaggcctgtataacgaactgcagaaagacaagatggccgaggcctacagcgagatcggcatgaagggcgagcggaggcggggcaagggccacgacggcctgtatcagggcctgtccaccgccaccaaggatacctacgacgccctgcacatgcaggccctgcccccaagg

SEQ ID NO: 115 - protein, 112 aa, Artificial Sequence
  CD3 Zeta
RVKFSRSADAPAYQQGQNQLYNELNLGRREEYDVLDKRRGRDPEMGGKPRRKNPQEGLYNELQKDKMAEAYSEIGMKGERRRGKGHDGLYQGLSTATKDTYDALHMQALPPR

SEQ ID NO: 116 - DNA, 126 bp, Unknown
  4-1BB
aaacggggcagaaagaaactcctgtatatattcaaacaaccatttatgagaccagtacaaactactcaagaggaagatggctgtagctgccgatttccagaagaagaagaaggaggatgtgaactg

SEQ ID NO: 117 - protein, 42 aa, Artificial Sequence
  4-1BB
KRGRKKLLYIFKQPFMRPVQTTQEEDGCSCRFPEEEEGGCEL

SEQ ID NO: 118 - DNA, 123 bp, Unknown
  CD28 cytoplasmic domain
cgcagcaagcggagcagaggcggccacagcgactacatgaacatgacccctagacggcctggccccaccagaaagcactaccagccctacgcccctccccgggactttgccgcctacagaagc

SEQ ID NO: 119 - protein, 41 aa, Artificial Sequence
  CD28 cytoplasmic domain
RSKRSRGGHSDYMNMTPRRPGPTRKHYQPYAPPRDFAAYRS

SEQ ID NO: 120 - DNA, 46 bp, Artificial Sequence
  DNA spacer
gctagcgtttaaacttaagcttggtaccgagctcggatccgccacc

SEQ ID NO: 121 - protein, 862 aa, Artificial Sequence
  HEA3(p65/S536E/K310Q) amino acid sequence variant
MVSKLSQLQTELLAALLESGLSKEALIQALGEPGPYLLAGEGPLDKGESCGGGRGELAELPNGLGETRGSEDETDDDGEDFTPPILKELENLSPEEAAHQKAVVETLLQEDPWRVAKMVKSYLQQHNIPQREVVDTTGLNQSHLSQHLNKGTPMKTQKRAALYTWYVRKQREVAQQFTHAGQGGLIEEPTGDELPTKKGRRNRFKWGPASQQILFQAYERQKNPSKEERETLVEECNRAECIQRGVSPSQAQGLGSNLVTEVRVYNWFANRRKEEAFRHKLSAGDMRAANLWPSPLMIKRSKKNSLALSLTADQMVSALLDAEPPILYSEYDPTRPFSEASMMGLLTNLADRELVHMINWAKRVPGFVDLTLHDQVHLLECAWLEILMIGLVWRSMEHPGKLLFAPNLLLDRNQGKCVEGMVEIFDMLLATSSRFRMMNLQGEEFVCLKSIILLNSGVYTFLSSTLKSLEEKDHIHRVLDKITDTLIHLMAKAGLTLQQQHQRLAQLLLILSHIRHMSNKRMEHLYSMKCKNVVPLYDLLLEMLDAHRLHAPTSRGGASVEETDQSHLATAGSTSSHSLQKYYITGEAEGFPATVEFQYLPDTDDRHRIEEKRKRTYETFQSIMKKSPFSGPTDPRPPPRRIAVPSRSSASVPKPAPQPYPFTSSLSTINYDEFPTMVFPSGQISQASALAPAPPQVLPQAPAPAPAPAMVSALAQAPAPVPVLAPGPPQAVAPPAPKPTQAGEGTLSEALLQLQFDDEDLGALLGNSTDPAVFTDLASVDNSEFQQLLNQGIPVAPHTTEPMLMEYPEAITRLVTGAQRPPDPAPAPLGAPGLPNGLLSGDEDFESIADMDFSALLSQISS

SEQ ID NO: 122 - DNA, 2586 bp, Artificial Sequence
  HEA3(p65/S536E/K310Q) variant nucleotide sequence
atggtgtccaagctgtcccagctgcagacagaactgctggcagcactgctggaaagcggcctgagcaaagaggccctgattcaggcactcggcgaacctggaccttatctgctcgctggcgaaggccctctggataagggcgagagctgtggcggaggaagaggagagctggccgagctgcctaacggcctgggcgagacaagaggcagcgaggacgagacagacgacgacggcgaggacttcaccccccccatcctgaaagagctggaaaacctgagccccgaggaagccgcccaccagaaagccgtggtggagacactgctgcaggaagatccctggcgggtcgccaagatggtcaagagctacctgcagcagcacaacatcccccagcgggaggtggtggacaccaccggcctgaaccagagccacctgagccagcacctgaacaagggcacccccatgaaaacccagaagagagccgccctgtacacttggtacgtgcggaagcagagagaggtggcccagcagtttacacacgccggccagggcggcctgatcgaggaacctaccggcgacgagctgcccaccaagaagggcagacggaaccggtttaagtggggccctgcatctcagcagatcctgttccaggcctacgagcggcagaagaaccccagcaaagaggaacgggagacactggtggaagagtgcaaccgggccgagtgcatccagagaggcgtgagcccttctcaggctcagggcctcggcagcaatctggtcaccgaagtgcgggtgtacaattggttcgccaaccggcggaaagaggaagccttccggcacaagctgtctgctggcgatatgagagccgccaacctgtggcccagccccctgatgatcaagcggagcaagaagaacagcctggccctgagcctgaccgccgatcagatggtgtccgctctgctggacgccgagccccctatcctgtacagcgagtacgaccccaccagacccttcagcgaggccagcatgatgggcctgctgaccaacctggccgaccgggagctggtgcacatgatcaactgggccaagcgggtgcccggcttcgtggacctgaccctgcacgaccaggtccacctgctggaatgtgcctggctggaaatcctgatgatcggcctcgtgtggagaagcatggaacaccccggcaagctgctgttcgcccccaacctgctcctggaccggaaccagggaaagtgcgtggagggcatggtggagatcttcgacatgctgctggccacctccagccggttccggatgatgaacctgcagggcgaggaattcgtgtgcctgaagtccatcatcctgctgaacagcggcgtgtacaccttcctgtcatccaccctgaagtccctggaagagaaggaccacatccaccgggtgctggacaagatcaccgacaccctgatccacctgatggccaaggctggcctgacactccagcagcagcaccagagactggcccagctgctgctgatcctgagccacatccggcacatgagcaacaagcggatggaacacctgtacagcatgaagtgcaagaacgtggtgcccctgtacgacctgctgctcgagatgctggatgcccacagactgcacgcccctacaagcagaggcggagccagcgtggaggaaaccgaccagtctcacctggccaccgccggcagcacaagcagccacagcctgcagaagtactacatcaccggcgaggccgagggattccctgccaccgtggagttccagtacctgcccgacaccgacgaccggcaccggatcgaggaaaagcggaagcggacctacgagacattccagagcatcatgaagaagtcccccttcagcggccccaccgatcccagacccccccctagaagaatcgccgtgcccagcagatctagcgccagcgtgcccaagcctgccccccagccctaccctttcaccagcagcctgagcaccatcaactacgacgagttccctaccatggtgttccccagcggccagatctctcaggcctctgctctggcacctgctccacctcaggtgctgcctcaggcccctgctccagccccagcccctgccatggtgtctgcactggcccaggctccagctcctgtgcctgtgctggcccctggacctcctcaggctgtggcccctcctgcccctaaacctacccaggccggggagggaacactgtctgaggccctgctgcagctccagttcgacgacgaggatctgggagcactgctgggcaatagcaccgaccccgccgtgtttaccgacctggcctccgtggacaacagcgagttccagcagctcctcaaccagggcatccctgtcgccccacacaccaccgagcccatgctgatggaataccccgaggccatcaccagactggtcacaggcgcccagaggcctccagatccagcaccagctccactgggagcccctggcctgcctaatgggctgctgtctggcgacgaggacttcgagagcattgccgacatggacttcagcgccctgctgtcccagatcagcagc

SEQ ID NO: 123 - protein, 142 aa, Artificial Sequence [sequence omitted]

SEQ ID NO: 124 - DNA, 426 bp, Artificial Sequence
  Survivin nucleotide sequence
atgggtgccccgacgttgccccctgcctggcagccctttctcaaggaccaccgcatctctacattcaagaactggcccttcttggagggctgcgcctgcaccccggagcggatggccgaggctggcttcatccactgccccactgagaacgagccagacttggcccagtgtttcttctgcttcaaggagctggaaggctgggagccagatgacgaccccatagaggaacataaaaagcattcgtccggttgcgctttcctttctgtcaagaagcagtttgaagaattaacccttggtgaatttttgaaactggacagagaaagagccaagaacaaaattgcaaaggaaaccaacaataagaagaaagaatttgaggaaactgtgaagaaagtgcgccgtgccatcgagcagctggctgcaatggat